European Patent Application EP 4 257 688 A1, published October 11, 2023. Title: NUCLEIC ACID CONSTRUCT FOR AIDS GENE THERAPY. Applicant: KANGLIN BIOTECH (HANGZHOU) CO., LTD. The sequence listing filed with the application follows.

SEQUENCE LISTING (28 sequences)

SEQ ID NO: 1 - protein, 744 aa, Artificial Sequence
MDMRVPAQLLGLLLLWLSGARCSELTQDPAVSVALKQTVTITCRGDSLRSHYASWYQKKPGQAPVLLFYGKNNRPSGIPDRFSGSASGNRASLTITGAQAEDEADYYCSSRDKSGSRLSVFGGGTKLTVLSQPKAAPSVTLFPPSSEELQANKATLVCLISDFYPGAVTVAWKADSSPVKAGVETTTPSKQSNNKYAASSYLSLTPEQWKSHRSYSCQVTHEGSTVEKTVAPTECSRKRRAPVKQTLNFDLLKLAGDVESNPGPMEFGLSWVFLVALFRGVQCEVRLRESGGGLVKPGGSLRLSCSASGFDFDNAWMTWVRQPPGKGLEWVGRITGPGEGWSVDYAESVKGRFTISRDNTKNTLYLEMNNVRTEDTGYYFCARTGKYYDFWFGYPPGEEYFQDWGQGTLVIVSSASTKGPSVFPLAPSSKSTSGGTAALGCLVKDYFPEPVTVSWNSGALTSGVHTFPAVLQSSGLYSLSSVVTVPSSSLGTQTYICNVNHKPSNTKVDKKVEPKSCDKTHTCPPCPAPELLGGPSVFLFPPKPKDTLMISRTPEVTCVVVDVSHEDPEVKFNWYVDGVEVHNAKTKPREEQYNSTYRVVSVLTVLHQDWLNGKEYKCKVSNKALPAPIEKTISKAKGQPREPQVYTLPPSRDELTKNQVSLTCLVKGFYPSDIAVEWESNGQPENNYKTTPPVLDSDGSFFLYSKLTVDKSRWQQGNVFSCSVMHEALHNHYTQKSLSLSPGK

SEQ ID NO: 2 - DNA, 2250 bp, Artificial Sequence
atggatatgagagtgcctgcccagctgctgggcctgctgctgctgtggctgagcggcgctagatgtagcgagctgacccaggatcccgccgtgagcgtggccctgaagcagaccgtgacaatcacctgcagaggcgatagcctgagatcccactacgccagctggtaccagaagaagcctggccaggcccccgtgctgctgttctacggcaagaacaatagacctagcggcatccctgacaggttctccggcagcgcctccggcaacagggcctctctgaccatcaccggcgcccaggccgaggacgaggctgattactactgttcctccagagacaagtccggctccagactgagcgtgttcggcggcggcaccaagctgacagtgctgagccagcctaaggccgcccctagcgtgacactgttccccccttccagcgaggagctgcaggccaataaggccacactggtgtgtctgatcagcgacttttaccctggcgccgtgacagtggcctggaaggccgattccagccccgtgaaggccggcgtggagacaaccacaccctccaagcagagcaacaataagtacgccgcctcctcctacctgtccctgacccccgagcagtggaagtcccacaggtcctactcctgtcaggtgacccacgagggcagcaccgtggagaagacagtggcccccaccgagtgttccagaaagaggagagcccctgtgaagcagaccctgaatttcgatctgctgaagctggccggcgacgtggagtccaatcccggcccaatggagttcggcctgagctgggtgtttctggtggccctgttcaggggcgtgcagtgcgaggtgagactgagggagagcggcggcggcctggtgaagcctggaggaagcctgagactgtcctgtagcgccagcggctttgactttgacaatgcctggatgacctgggtgagacagcctcctggcaagggcctggagtgggtgggcagaatcaccggccccggcgagggatggtccgtggattacgccgagagcgtgaagggcagattcactatcagcagggataatacaaagaatacactgtacctggagatgaacaacgtgaggaccgaggacaccggctactacttctgtgccaggaccggcaagtactacgatttctggttcggctacccccctggcgaggagtactttcaggactggggccagggcacactggtcattgtgagctccgcctccaccaagggcccaagcgtgttccctctggccccttccagcaagagcacctccggcggcaccgccgccctgggctgtctggtgaaggactacttccccgagcctgtgaccgtgtcctggaatagcggcgccctgacctccggcgtgcacacctttcctgccgtgctgcagagctccggcctgtacagcctgtccagcgtggtgaccgtgcctagctccagcctgggcacccagacctacatctgcaatgtgaaccacaagccatccaacaccaaggtggacaagaaggtggagcccaagtcctgcgacaagacccacacctgcccaccttgccccgcccctgagctgctgggcggccctagcgtgttcctgtttccacccaagcctaaggataccctgatgatctcccgcacccctgaggtgacctgcgtggtggtggatgtgagccacgaggacccagaggtgaagttcaattggtacgtggacggcgtggaggtgcacaacgccaagaccaagccccgggaggagcagtacaactccacctaccgggtggtgtccgtgctgaccgtgctgcaccaggactggctgaacggcaaggagtacaagtgtaaggtgtccaacaaggccctgcccgccccaatcgagaagaccatcagcaaggccaagggccagcctagagagccccaggtgtacaccctgcccccatcccgcgacgagctgaccaagaaccaggtgtccctgacctgcctggtgaagggcttctacccaagcgatatcgccgtggagtgggagagcaacggccagccagagaataactacaagaccacccctcccgtgctggacagcgacggctcctttttcctgtactccaagctgaccgtggacaagtcccggtggcagcagggcaacgtgttcagctgctccgtgatgcacgaggccctgcacaaccactacacccagaagtccctgagcctgagccccggcaagagaaagaggcgggcccca

SEQ ID NO: 3 - protein, 745 aa, Artificial Sequence
MDMRVPAQLLGLLLLWLSGARCQSALTQPPSASGSPGQSITISCTGTSNNFVSWYQQHAGKAPKLVIYDVNKRPSGVPDRFSGSKSGNTASLTVSGLQTDDEAVYYCGSLVGNWDVIFGGGTKLTVLGQPKAAPSVTLFPPSSEELQANKATLVCLISDFYPGAVTVAWKADSSPVKAGVETTTPSKQSNNKYAASSYLSLTPEQWKSHRSYSCQVTHEGSTVEKTVAPTECSRKRRAPVKQTLNFDLLKLAGDVESNPGPMEFGLSWVFLVALFRGVQCQPQLQESGPTLVEASETLSLTCAVSGDSTAACNSFWGWVRQPPGKGLEWVGSLSHCASYWNRGWTYHNPSLKSRLTLALDTPKNLVFLKLNSVTAADTATYYCARFGGEVLRYTDWPKPAWVDLWGRGTLVTVSSASTKGPSVFPLAPSSKSTSGGTAALGCLVKDYFPEPVTVSWNSGALTSGVHTFPAVLQSSGLYSLSSVVTVPSSSLGTQTYICNVNHKPSNTKVDKRVEPKSCDKTHTCPPCPAPELLGGPSVFLFPPKPKDTLMISRTPEVTCVVVDVSHEDPEVKFNWYVDGVEVHNAKTKPREEQYNSTYRVVSVLTVLHQDWLNGKEYKCKVSNKALPAPIEKTISKAKGQPREPQVYTLPPSRDELTKNQVSLTCLVKGFYPSDIAVEWESNGQPENNYKTTPPVLDSDGSFFLYSKLTVDKSRWQQGNVFSCSVMHEALHNHYTQKSLSLSPGK

SEQ ID NO: 4 - DNA, 2256 bp, Artificial Sequence
atggacatgagggtgcccgcccagctgctgggcctgctgctgctgtggctgagcggcgctaggtgccagagcgccctgacccagccccctagcgcttccggaagccctggccagtccatcaccatcagctgtaccggcaccagcaacaactttgtgagctggtaccagcagcacgccggcaaggcccctaagctggtcatctatgatgtgaataagaggccttccggcgtgcccgacaggttcagcggcagcaagtccggcaataccgcctccctgacagtgtccggcctgcagaccgatgacgaggccgtgtactactgcggcagcctggtgggcaattgggacgtgatcttcggcggcggcacaaagctgacagtgctgggccagcccaaggccgccccttctgtgaccctgttcccccctagctccgaggagctgcaggccaataaggccaccctggtgtgtctgatcagcgatttctaccccggcgccgtgaccgtggcctggaaggctgacagcagccccgtgaaggccggcgtggagaccaccacaccctccaagcagagcaataacaagtacgccgcctcctcctacctgtccctgacccctgagcagtggaagagccacaggtcctacagctgccaggtgacccacgagggcagcaccgtggagaagacagtggcccccaccgagtgttccaggaagagaagagcccctgtgaagcagaccctgaacttcgatctgctgaagctggccggcgacgtggagagcaaccctggccctatggagtttggcctgtcctgggtgttcctggtggccctgtttagaggcgtgcagtgtcagcctcagctgcaggagagcggccctaccctggtggaggccagcgagaccctgtccctgacatgcgccgtgtccggcgatagcacagccgcctgcaactccttttggggctgggtgagacagccccccggcaagggactggagtgggtgggatccctgagccactgtgcctcctactggaataggggctggacctaccacaaccctagcctgaagtccagactgacactggccctggatacacccaagaacctggtgttcctgaagctgaactccgtgacagccgccgataccgccacctactactgtgccagattcggcggcgaggtgctgagatacacagactggcccaagcccgcctgggtggatctgtggggcagaggcaccctggtgacagtgagctccgcctccaccaagggcccaagcgtgttccctctggccccttccagcaagagcacctccggcggcaccgccgccctgggctgtctggtgaaggactacttccccgagcctgtgaccgtgtcctggaatagcggcgccctgacctccggcgtgcacacctttcctgccgtgctgcagagctccggcctgtacagcctgtccagcgtggtgaccgtgcctagctccagcctgggcacccagacctacatctgcaatgtgaaccacaagccatccaacaccaaggtggacaagaaggtggagcccaagtcctgcgacaagacccacacctgcccaccttgccccgcccctgagctgctgggcggccctagcgtgttcctgtttccacccaagcctaaggataccctgatgatctcccgcacccctgaggtgacctgcgtggtggtggatgtgagccacgaggacccagaggtgaagttcaattggtacgtggacggcgtggaggtgcacaacgccaagaccaagccccgggaggagcagtacaactccacctaccgggtggtgtccgtgctgaccgtgctgcaccaggactggctgaacggcaaggagtacaagtgtaaggtgtccaacaaggccctgcccgccccaatcgagaagaccatcagcaaggccaagggccagcctagagagccccaggtgtacaccctgcccccatcccgcgacgagctgaccaagaaccaggtgtccctgacctgcctggtgaagggcttctacccaagcgatatcgccgtggagtgggagagcaacggccagccagagaataactacaagaccacccctcccgtgctggacagcgacggctcctttttcctgtactccaagctgaccgtggacaagtcccggtggcagcagggcaacgtgttcagctgctccgtgatgcacgaggccctgcacaaccactacacccagaagtccctgagcctgagccccggcaagagaaagaggcgggccccatga

SEQ ID NO: 5 - protein, 786 aa, Artificial Sequence
MDAMKRGLCCVLLLCGAVFVSPSELTQDPAVSVALKQTVTITCRGDSLRSHYASWYQKKPGQAPVLLFYGKNNRPSGIPDRFSGSASGNRASLTITGAQAEDEADYYCSSRDKSGSRLSVFGGGTKLTVLGGGGSGGGGSGGGGSEVRLRESGGGLVKPGGSLRLSCSASGFDFDNAWMTWVRQPPGKGLEWVGRITGPGEGWSVDYAESVKGRFTISRDNTKNTLYLEMNNVRTEDTGYYFCARTGKYYDFWFGYPPGEEYFQDWGQGTLVIVSSGGGGSGGGGSGGGGSGGGGSGGGGSDIVMTQSPDSLAVSLGERVTMNCKSSQSLLYSTNQKNYLAWYQQKPGQSPKLLIYWASTRESGVPDRFSGSGSGTDFTLTISSVQAEDVAVYYCQQYYSYRTFGGGTKLEIKRTVAGGGGSGGGGSGGGGSQVQLQQSGPEVVKPGASVKMSCKASGYTFTSYVIHWVRQKPGQGLDWIGYINPYNDGTDYDEKFKGKATLTSDTSTSTAYMELSSLRSEDTAVYYCAREKDNYATGAWFAYWGQGTLVTVSSEPKSCDKTHTCPPCPAPELLGGPSVFLFPPKPKDTLMISRTPEVTCVVVDVSHEDPEVKFNWYVDGVEVHNAKTKPREEQYNSTYRVVSVLTVLHQDWLNGKEYKCKVSNKALPAPIEKTISKAKGQPREPQVYTLPPSRDELTKNQVSLTCLVKGFYPSDIAVEWESNGQPENNYKTTPPVLDSDGSFFLYSKLTVDKSRWQQGNVFSCSVMHEALHNHYTQKSLSLSPGK

SEQ ID NO: 6 - DNA, 2361 bp, Artificial Sequence
atggatgcaatgaagagagggctctgctgtgtgctgctgctgtgtggagcagtcttcgtttcgcccagcgagctgacacaggaccctgccgtgtccgtggccctgaagcagaccgtgacaatcacctgcagaggcgattccctgagatcccactacgcctcctggtaccagaagaagcctggccaggcccccgtgctgctgttttacggcaagaataaccgccccagcggcatccccgatagattttccggcagcgcctccggcaacagagccagcctgacaatcaccggcgcccaggccgaggacgaggctgattactactgcagctccagagataagagcggcagcagactgtccgtgtttggcggcggcaccaagctgaccgtgctcggaggaggaggaagcggaggaggaggctcaggcggcggcggctctgaggtgaggctgagagagtccggcggcggcctggtgaagcccggaggatctctgaggctgtcctgctccgcctccggcttcgattttgacaatgcctggatgacctgggtgagacagccccctggcaagggcctggagtgggtgggaaggatcacaggccccggcgagggctggtccgtggattacgccgagtccgtgaagggcaggttcacaatctccagggataacaccaagaacaccctgtacctggagatgaacaacgtgaggacagaggataccggctactacttttgcgccagaacaggcaagtactacgacttttggttcggctacccccctggcgaggagtacttccaggattggggccagggcaccctggtcattgtgtccagcggcggcggcggcagtggcggcggcggaagcggcggcggcggctctggcggcggcggcagcggcggcggcggctccgacatcgtgatgacccagtctcctgatagcctggccgtgagcctgggcgagagagtgacaatgaactgtaagtctagccagagcctgctgtactccaccaaccagaagaattacctggcctggtatcagcagaagcctggccagtccccaaagctgctgatctattgggcatctacaagggagagcggagtgccagacagattcagcggatccggatctggaaccgacttcaccctgacaatctcctctgtgcaggccgaggacgtggccgtgtactattgccagcagtactatagctacaggacattcggcggcggcaccaagctggagatcaagcgcaccgtggccggaggaggaggatctggcggaggagggtccggcggcggcggctcccaggtgcagctgcagcagagcggaccagaggtggtgaagcctggagcctccgtgaagatgtcttgtaaggccagcggctacaccttcacatcctatgtgatccactgggtgaggcagaagccaggacagggactggactggatcggctacatcaacccttataatgatggcaccgactacgatgagaagtttaagggcaaggccaccctgacatccgataccagcacatccaccgcctatatggagctgagctccctgcggtctgaggacacagccgtgtactattgcgccagagagaaggataactacgcaaccggagcatggttcgcatattggggacagggtaccctggtcaccgtgtctagcgagcccaagagctgtgacaagacacacacctgccctccatgtccagcaccagagctgctgggagggccctccgtgttcctgtttccccctaagccaaaggatacactgatgatctccaggacaccagaggtgacctgcgtggtggtggacgtgtctcacgaggatcctgaggtgaagtttaactggtacgtggacggcgtggaggtgcacaatgccaagaccaagcctagggaggagcagtacaattctacatatcgcgtggtgagcgtgctgaccgtgctgcaccaggattggctgaacggcaaggagtataagtgcaaggtgagcaataaggccctgcctgccccaatcgagaagacaatctccaaggcaaagggacagccaagggagcctcaggtgtacaccctgccaccctctcgcgacgagctgacaaagaaccaggtgagcctgacctgtctggtgaagggcttctatcctagcgatattgccgtggagtgggagtccaatggccagccagagaacaattacaagaccacacctccagtgctggactccgatggctctttctttctgtattccaagctgacagtggacaagtctagatggcagcagggcaacgtgttttcttgtagcgtgatgcacgaggccctgcacaatcactacacccagaagtccctgtctctgagccccggcaagtag

SEQ ID NO: 7 - protein, 787 aa, Artificial Sequence
MDAMKRGLCCVLLLCGAVFVSPQSALTQPPSASGSPGQSITISCTGTSNNFVSWYQQHAGKAPKLVIYDVNKRPSGVPDRFSGSKSGNTASLTVSGLQTDDEAVYYCGSLVGNWDVIFGGGTKLTVLGGGGSGGGGSGGGGSQPQLQESGPTLVEASETLSLTCAVSGDSTAACNSFWGWVRQPPGKGLEWVGSLSHCASYWNRGWTYHNPSLKSRLTLALDTPKNLVFLKLNSVTAADTATYYCARFGGEVLRYTDWPKPAWVDLWGRGTLVTVSSGGGGSGGGGSGGGGSGGGGSGGGGSDIVMTQSPDSLAVSLGERVTMNCKSSQSLLYSTNQKNYLAWYQQKPGQSPKLLIYWASTRESGVPDRFSGSGSGTDFTLTISSVQAEDVAVYYCQQYYSYRTFGGGTKLEIKRTVAGGGGSGGGGSGGGGSQVQLQQSGPEVVKPGASVKMSCKASGYTFTSYVIHWVRQKPGQGLDWIGYINPYNDGTDYDEKFKGKATLTSDTSTSTAYMELSSLRSEDTAVYYCAREKDNYATGAWFAYWGQGTLVTVSSEPKSCDKTHTCPPCPAPELLGGPSVFLFPPKPKDTLMISRTPEVTCVVVDVSHEDPEVKFNWYVDGVEVHNAKTKPREEQYNSTYRVVSVLTVLHQDWLNGKEYKCKVSNKALPAPIEKTISKAKGQPREPQVYTLPPSRDELTKNQVSLTCLVKGFYPSDIAVEWESNGQPENNYKTTPPVLDSDGSFFLYSKLTVDKSRWQQGNVFSCSVMHEALHNHYTQKSLSLSPGK

SEQ ID NO: 8 - DNA, 2364 bp, Artificial Sequence
atggatgcaatgaagagagggctctgctgtgtgctgctgctgtgtggagcagtcttcgtttcgccccagagcgccctgacacagccaccttccgcctctggaagcccaggacagagcatcaccatctcctgtaccggcacatccaacaatttcgtgtcttggtatcagcagcacgcaggcaaggcaccaaagctggtcatctacgacgtgaacaagcggccaagcggcgtgcccgatagattttccggctctaagagcggcaatacagcctctctgaccgtgagcggcctgcagaccgacgatgaggccgtgtactattgcggctccctggtgggcaactgggacgtgatcttcggcggcggcacaaagctgaccgtgctgggaggaggaggaagcggaggaggaggctcaggcggcggcggctctcagccacagctgcaggagagcggacccacactggtggaggcatccgagacactgtctctgacctgcgccgtgtccggcgattctaccgcagcctgtaatagcttttggggatgggtgcggcagccaccaggcaagggcctggagtgggtgggctccctgtctcactgcgcctcctactggaaccggggctggacctatcacaatccaagcctgaagtccagactgacactggccctggacacccccaagaacctggtgttcctgaagctgaatagcgtgacagccgccgataccgccacatactattgtgccaggtttggaggagaggtgctgaggtacaccgactggcccaagcctgcatgggtggatctgtggggaaggggcacactggtgaccgtgagctccggcggcggcggcagtggcggcggcggaagcggcggcggcggctctggcggcggcggcagcggcggcggcggctccgacatcgtgatgacccagtctcctgatagcctggccgtgagcctgggcgagagagtgacaatgaactgtaagtctagccagagcctgctgtactccaccaaccagaagaattacctggcctggtatcagcagaagcctggccagtccccaaagctgctgatctattgggcatctacaagggagagcggagtgccagacagattcagcggatccggatctggaaccgacttcaccctgacaatctcctctgtgcaggccgaggacgtggccgtgtactattgccagcagtactatagctacaggacattcggcggcggcaccaagctggagatcaagcgcaccgtggccggaggaggaggatctggcggaggagggtccggcggcggcggctcccaggtgcagctgcagcagagcggaccagaggtggtgaagcctggagcctccgtgaagatgtcttgtaaggccagcggctacaccttcacatcctatgtgatccactgggtgaggcagaagccaggacagggactggactggatcggctacatcaacccttataatgatggcaccgactacgatgagaagtttaagggcaaggccaccctgacatccgataccagcacatccaccgcctatatggagctgagctccctgcggtctgaggacacagccgtgtactattgcgccagagagaaggataactacgcaaccggagcatggttcgcatattggggacagggtaccctggtcaccgtgtctagcgagcccaagagctgtgacaagacacacacctgccctccatgtccagcaccagagctgctgggagggccctccgtgttcctgtttccccctaagccaaaggatacactgatgatctccaggacaccagaggtgacctgcgtggtggtggacgtgtctcacgaggatcctgaggtgaagtttaactggtacgtggacggcgtggaggtgcacaatgccaagaccaagcctagggaggagcagtacaattctacatatcgcgtggtgagcgtgctgaccgtgctgcaccaggattggctgaacggcaaggagtataagtgcaaggtgagcaataaggccctgcctgccccaatcgagaagacaatctccaaggcaaagggacagccaagggagcctcaggtgtacaccctgccaccctctcgcgacgagctgacaaagaaccaggtgagcctgacctgtctggtgaagggcttctatcctagcgatattgccgtggagtgggagtccaatggccagccagagaacaattacaagaccacacctccagtgctggactccgatggctctttctttctgtattccaagctgacagtggacaagtctagatggcagcagggcaacgtgttttcttgtagcgtgatgcacgaggccctgcacaatcactacacccagaagtccctgtctctgagccccggcaagtag

SEQ ID NO: 9 - DNA, 7128 bp, Artificial Sequence
ggccgcgttgctggcgtttttccataggctccgcccccctgacgagcatcacaaaaatcgacgctcaagtcagaggtggcgaaacccgacaggactataaagataccaggcgtttccccctggaagctccctcgtgcgctctcctgttccgaccctgccgcttaccggatacctgtccgcctttctcccttcgggaagcgtggcgctttctcatagctcacgctgtaggtatctcagttcggtgtaggtcgttcgctccaagctgggctgtgtgcacgaaccccccgttcagcccgaccgctgcgccttatccggtaactatcgtcttgagtccaacccggtaagacacgacttatcgccactggcagcagccactggtaacaggattagcagagcgaggtatgtaggcggtgctacagagttcttgaagtggtggcctaactacggctacactagaagaacagtatttggtatctgcgctctgctgaagccagttaccttcggaaaaagagttggtagctcttgatccggcaaacaaaccaccgctggtagcggtggtttttttgtttgcaagcagcagattacgcgcagaaaaaaaggatctcaagaagatcctttgatcttttctacggggtctgacgctcagtggaacgaaaactcacgttaagggattttggtcatgaagcgcttttgaagctcggatccgaacaaacgacccaacacccgtgcgttttattctgtctttttattgccgatcccctcagaagaactcgtcaagaaggcgatagaaggcgatgcgctgcgaatcgggagcggcgataccgtaaagcacgaggaagcggtcagcccattcgccgccaagctcttcagcaatatcacgggtagccaacgctatgtcctgatagcggtccgccacacccagccggccacagtcgatgaatccagaaaagcggccattttccaccatgatattcggcaagcaggcatcgccatgggtcacgacgagatcctcgccgtcgggcatgctcgccttgagcctggcgaacagttcggctggcgcgagcccctgatgctcttcgtccagatcatcctgatcgacaagaccggcttccatccgagtacgtgctcgctcgatgcgatgtttcgcttggtggtcgaatgggcaggtagccggatcaagcgtatgcagccgccgcattgcatcagccatgatggatactttctcggcaggagcaaggtgagatgacaggagatcctgccccggcacttcgcccaatagcagccagtcccttcccgcttcagtgacaacgtcgagcacagctgcgcaaggaacgcccgtcgtggccagccacgatagccgcgctgcctcgtcttgcagttcattcagggcaccggacaggtcggtcttgacaaaaagaaccgggcgcccctgcgctgacagccggaacacggcggcatcagagcagccgattgtctgttgtgcccagtcatagccgaatagcctctccacccaagcggccggagaacctgcgtgcaatccatcttgttcaatcatgcgaaacgatcctcatcctgtctcttgatcagagcttgatcccctgcgccatcagatccttggcggcaagaaagccatccagtttactttgcagggcttcccaaccttaccagaggcctgcgccgcggccagctggctagcaattcccgggttaactctagagacattgattattgactagttattaatagtaatcaattacggggtcattagttcatagcccatatatggagttccgcgttacataacttacggtaaatggcccgcctggctgaccgcccaacgacccccgcccattgacgtcaataatgacgtatgttcccatagtaacgccaatagggactttccattgacgtcaatgggtggagtatttacggtaaactgcccacttggcagtacatcaagtgtatcatatgccaagtacgccccctattgacgtcaatgacggtaaatggcccgcctggcattatgcccagtacatgaccttatgggactttcctacttggcagtacatctacgtattagtcatcgctattaccatggtgatgcggttttggcagtacatcaatgggcgtggatagcggtttgactcacggggatttccaagtctccaccccattgacgtcaatgggagtttgttttggcaccaaaatcaacgggactttccaaaatgtcgtaacaactccgccccattgacgcaaatgggcggtaggcgtgtacggtgggaggtctatataagcagagctcgtttagtgaaccggggtctctctggttagaccagatctgagcctgggagctctctggctaactagggaacccactgcttaagcctcaataaagcttgccttgagtgcttcaagtagtgtgtgcccgtctgttgtgtgactctggtaactagagatccctcagacccttttagtcagtgtggaaaatctctagcagtggcgcccgaacagggacttgaaagcgaaagggaaaccagaggagctctctcgacgcaggactcggcttgctgaagcgcgcacggcaagaggcgaggggcggcgactggtgagtacgccaaaaattttgactagcggaggctagaaggagagagatgggtgcgagagcgtcagtattaagcgggggagaattagatcgcgatgggaaaaaattcggttaaggccagggggaaagaaaaaatataaattaaaacatatagtatgggcaagcagggagctagaacgattcgcagttaatcctggcctgttagaaacatcagaaggctgtagacaaatactgggacagctacaaccatcccttcagacaggatcagaagaacttagatcattatataatacagtagcaaccctctattgtgtgcatcaaaggatagagataaaagacaccaaggaagctttagacaagatagaggaagagcaaaacaaaagtaagaccaccgcacagcaagcggccgctgatcttcagacctggaggaggagatatgagggacaattggagaagtgaattatataaatataaagtagtaaaaattgaaccattaggagtagcacccaccaaggcaaagagaagagtggtgcagagagaaaaaagagcagtgggaataggagctttgttccttgggttcttgggagcagcaggaagcactatgggcgcagcgtcaatgacgctgacggtacaggccagacaattattgtctggtatagtgcagcagcagaacaatttgctgagggctattgaggcgcaacagcatctgttgcaactcacagtctggggcatcaagcagctccaggcaagaatcctggctgtggaaagatacctaaaggatcaacagctcctggggatttggggttgctctggaaaactcatttgcaccactgctgtgccttggaatgctagttggagtaataaatctctggaacagatttggaatcacacgacctggatggagtgggacagagaaattaacaattacacaagcttaatacactccttaattgaagaatcgcaaaaccagcaagaaaagaatgaacaagaattattggaattagataaatgggcaagtttgtggaattggtttaacataacaaattggctgtggtatataaaattattcataatgatagtaggaggcttggtaggtttaagaatagtttttgctgtactttctatagtgaatagagttaggcagggatattcaccattatcgtttcagacccacctcccaaccccgaggggacccgacaggcccgaaggaatagaagaagaaggtggagagagagacagagacagatccattcgattagtgaacggatctcgacggtatcggttaacttttaaaagaaaaggggggattggggggtacagtgcaggggaaagaatagtagacataatagcaacagacatacaaactaaagaattacaaaaacaaattacaaaaattcaaaattttatcgatcacgagactagcctcgaggcatgcctgcaggaattcgctccggtgcccgtcagtgggcagagcgcacatcgcccacagtccccgagaagttggggggaggggtcggcaattgaaccggtgcctagagaaggtggcgcggggtaaactgggaaagtgatgtcgtgtactggctccgcctttttcccgagggtgggggagaaccgtatataagtgcagtagtcgccgtgaacgttctttttcgcaacgggtttgccgccagaacacaggtaagtgccgtgtgtggttcccgcgggcctggcctctttacgggttatggcccttgcgtgccttgaattacttccacgcccctggctgcagtacgtgattcttgatcccgagcttcgggttggaagtgggtgggagagttcgaggccttgcgcttaaggagccccttcgcctcgtgcttgagttgaggcctggcttgggcgctggggccgccgcgtgcgaatctggtggcaccttcgcgcctgtctcgctgctttcgataagtctctagccatttaaaatttttgatgacctgctgcgacgctttttttctggcaagatagtcttgtaaatgcgggccaagatctgcacactggtatttcggtttttggggccgcgggcggcgacggggcccgtgcgtcccagcgcacatgttcggcgaggcggggcctgcgagcgcggccaccgagaatcggacgggggtagtctcaagctggccggcctgctctggtgcctggcctcgcgccgccgtgtatcgccccgccctgggcggcaaggctggcccggtcggcaccagttgcgtgagcggaaagatggccgcttcccggccctgctgcagggagctcaaaatggaggacgcggcgctcgggagagcgggcgggtgagtcacccacacaaaggaaaagggcctttccgtcctcagccgtcgcttcatgtgactccacggagtaccgggcgccgtccaggcacctcgattagttctcgagcttttggagtacgtcgtctttaggttggggggaggggttttatgcgatggagtttccccacactgagtgggtggagactgaagttaggccagcttggcacttgatgtaattctccttggaatttgccctttttgagtttggatcttggttcattctcaagcctcagacagtggttcaaagtttttttcttccatttcaggtgtcgtgaggatctatttccggtgagacccaagctggctagctaaacttacgcgtgcctcggatcctccagtgtggtgtgcagatatccagcacagtcccgggccgagtctagacgtttaaacccgctgatcaggtcgacaatcaacctctggattacaaaatttgtgaaagattgactggtattcttaactatgttgctccttttacgctatgtggatacgctgctttaatgcctttgtatcatgctattgcttcccgtatggctttcattttctcctccttgtataaatcctggttgctgtctctttatgaggagttgtggcccgttgtcaggcaacgtggcgtggtgtgcactgtgtttgctgacgcaacccccactggttggggcattgccaccacctgtcagctcctttccgggactttcgctttccccctccctattgccacggcggaactcatcgccgcctgccttgcccgctgctggacaggggctcggctgttgggcactgacaattccgtggtgttgtcggggaagctgacgtcctttccatggctgctcgcctgtgttgccacctggattctgcgcgggacgtccttctgctacgtcccttcggccctcaatccagcggaccttccttcccgcggcctgctgccggctctgcggcctcttccgcgtcttcgccttcgccctcagacgagtcggatctccctttgggccgcctccccgcggtacctttaagaccaatgacttacaaggcagctgtagatcttagccactttttaaaagaaaaggggggactggaagggctaattcactcccaacgaagacaagatctgctttttgcttgtactgggtctctctggttagaccagatctgagcctgggagctctctggctaactagggaacccactgcttaagcctcaataaagcttgccttgagtgcttcaagtagtgtgtgcccgtctgttgtgtgactctggtaactagagatccctcagacccttttagtcagtgtggaaaatctctagcagtagtagttcatgtcatcttattattcagtatttataacttgcaaagaaatgaatatcagagagtgagaggaacttgtttattgcagcttataatggttacaaataaagcaatagcatcacaaatttcacaaataaagcatttttttcactgcattctagttgtggtttgtccaaactcatcaatgtatcttatcatgtctggctctagctatcccgcccctaactccgcccatcccgcccctaactccgcccagttccgcccattctccgccccatggctgactaattttttttatttatgcagaggccgaggccgcctcggcctctgagctattccagaagtagtgaggaggcttttttggaggccgctagcgtcgaccattacttattgttttagctgtcctcatgaatgtcttttcactacccatttgcttatcctgcatctctcagccttgactccactcagttctcttgcttagagataccacctttcccctgaagtgttccttccatgttttacggcgagatggtttctcctcgcctggccactcagccttagttgtctctgttgtcttatagaggtctacttgaagaaggaaaaacagggggcatggtttgactgtcctgtgagcccttcttccctgcctcccccactcacagtgacccggaatccctcgacatggcagtctagcactagtgcggccgcagatctgcttcctcgctcactgactcgctgcgctcggtcgttcggctgcggcgagcggtatcagctcactcaaaggcggtaatacggttatccacagaatcaggggataacgcaggaaagaacatgtgagcaaaaggccagcaaaaggccaggaaccgtaaaaa

SEQ ID NO: 10 - DNA, 814 bp, Artificial Sequence
cgttacataacttacggtaaatggcccgcctggctgaccgcccaacgacccccgcccattgacgtcaataatgacgtatgttcccatagtaacgccaatagggactttccattgacgtcaatgggtggagtatttacggtaaactgcccacttggcagtacatcaagtgtatcatatgccaagtacgccccctattgacgtcaatgacggtaaatggcccgcctggcattatgcccagtacatgaccttatgggactttcctacttggcagtacatctacgtattagtcatcgctattaccatggtcgaggtgagccccacgttctgcttcactctccccatctcccccccctccccacccccaattttgtatttatttattttttaattattttgtgcagcgatgggggcggggggggggggggggcgcgcgccaggcggggcggggcggggcgaggggcggggcggggcgaggcggagaggtgcggcggcagccaatcagagcggcgcgctccgaaagtttccttttatggcgaggcggcggcggcggcggccctataaaaagcgaagcgcgcggcgggcgggagtcgctgcgacgctgccttcgccccgtgccccgctccgccgccgcctcgcgccgcccgccccggctctgactgaccgcgttactcccacaggtgagcgggcgggacggcccttctcctccgggctgtaattagctgagcaagaggtaagggtttaagggatggttggttggtggggtattaatgtttaattacctggagcacctgcctgaaatcactttttttcaggt

SEQ ID NO: 11 - DNA, 9068 bp, Artificial Sequence
ggccgcgttgctggcgtttttccataggctccgcccccctgacgagcatcacaaaaatcgacgctcaagtcagaggtggcgaaacccgacaggactataaagataccaggcgtttccccctggaagctccctcgtgcgctctcctgttccgaccctgccgcttaccggatacctgtccgcctttctcccttcgggaagcgtggcgctttctcatagctcacgctgtaggtatctcagttcggtgtaggtcgttcgctccaagctgggctgtgtgcacgaaccccccgttcagcccgaccgctgcgccttatccggtaactatcgtcttgagtccaacccggtaagacacgacttatcgccactggcagcagccactggtaacaggattagcagagcgaggtatgtaggcggtgctacagagttcttgaagtggtggcctaactacggctacactagaagaacagtatttggtatctgcgctctgctgaagccagttaccttcggaaaaagagttggtagctcttgatccggcaaacaaaccaccgctggtagcggtggtttttttgtttgcaagcagcagattacgcgcagaaaaaaaggatctcaagaagatcctttgatcttttctacggggtctgacgctcagtggaacgaaaactcacgttaagggattttggtcatgaagcgcttttgaagctcggatccgaacaaacgacccaacacccgtgcgttttattctgtctttttattgccgatcccctcagaagaactcgtcaagaaggcgatagaaggcgatgcgctgcgaatcgggagcggcgataccgtaaagcacgaggaagcggtcagcccattcgccgccaagctcttcagcaatatcacgggtagccaacgctatgtcctgatagcggtccgccacacccagccggccacagtcgatgaatccagaaaagcggccattttccaccatgatattcggcaagcaggcatcgccatgggtcacgacgagatcctcgccgtcgggcatgctcgccttgagcctggcgaacagttcggctggcgcgagcccctgatgctcttcgtccagatcatcctgatcgacaagaccggcttccatccgagtacgtgctcgctcgatgcgatgtttcgcttggtggtcgaatgggcaggtagccggatcaagcgtatgcagccgccgcattgcatcagccatgatggatactttctcggcaggagcaaggtgagatgacaggagatcctgccccggcacttcgcccaatagcagccagtcccttcccgcttcagtgacaacgtcgagcacagctgcgcaaggaacgcccgtcgtggccagccacgatagccgcgctgcctcgtcttgcagttcattcagggcaccggacaggtcggtcttgacaaaaagaaccgggcgcccctgcgctgacagccggaacacggcggcatcagagcagccgattgtctgttgtgcccagtcatagccgaatagcctctccacccaagcggccggagaacctgcgtgcaatccatcttgttcaatcatgcgaaacgatcctcatcctgtctcttgatcagagcttgatcccctgcgccatcagatccttggcggcaagaaagccatccagtttactttgcagggcttcccaaccttaccagaggcctgcgccgcggccagctggctagcaattcccgggttaactctagagacattgattattgactagttattaatagtaatcaattacggggtcattagttcatagcccatatatggagttccgcgttacataacttacggtaaatggcccgcctggctgaccgcccaacgacccccgcccattgacgtcaataatgacgtatgttcccatagtaacgccaatagggactttccattgacgtcaatgggtggagtatttacggtaaactgcccacttggcagtacatcaagtgtatcatatgccaagtacgccccctattgacgtcaatgacggtaaatggcccgcctggcattatgcccagtacatgaccttatgggactttcctacttggcagtacatctacgtattagtcatcgctattaccatggtgatgcggttttggcagtacatcaatgggcgtggatagcggtttgactcacggggatttccaagtctccaccccattgacgtcaatgggagtttgttttggcaccaaaatcaacgggactttccaaaatgtcgtaacaactccgccccattgacgcaaatgggcggtaggcgtgtacggtgggaggtctatataagcagagctcgtttagtgaaccggggtctctctggttagaccagatctgagcctgggagctctctggctaactagggaacccactgcttaagcctcaataaagcttgccttgagtgcttcaagtagtgtgtgcccgtctgttgtgtgactctggtaactagagatccctcagacccttttagtcagtgtggaaaatctctagcagtggcgcccgaacagggacttgaaagcgaaagggaaaccagaggagctctctcgacgcaggactcggcttgctgaagcgcgcacggcaagaggcgaggggcggcgactggtgagtacgccaaaaattttgactagcggaggctagaaggagagagatgggtgcgagagcgtcagtattaagcgggggagaattagatcgcgatgggaaaaaattcggttaaggccagggggaaagaaaaaatataaattaaaacatatagtatgggcaagcagggagctagaacgattcgcagttaatcctggcctgttagaaacatcagaaggctgtagacaaatactgggacagctacaaccatcccttcagacaggatcagaagaacttagatcattatataatacagtagcaaccctctattgtgtgcatcaaaggatagagataaaagacaccaaggaagctttagacaagatagaggaagagcaaaacaaaagtaagaccaccgcacagcaagcggccgctgatcttcagacctggaggaggagatatgagggacaattggagaagtgaattatataaatataaagtagtaaaaattgaaccattaggagtagcacccaccaaggcaaagagaagagtggtgcagagagaaaaaagagcagtgggaataggagctttgttccttgggttcttgggagcagcaggaagcactatgggcgcagcgtcaatgacgctgacggtacaggccagacaattattgtctggtatagtgcagcagcagaacaatttgctgagggctattgaggcgcaacagcatctgttgcaactcacagtctggggcatcaagcagctccaggcaagaatcctggctgtggaaagatacctaaaggatcaacagctcctggggatttggggttgctctggaaaactcatttgcaccactgctgtgccttggaatgctagttggagtaataaatctctggaacagatttggaatcacacgacctggatggagtgggacagagaaattaacaattacacaagcttaatacactccttaattgaagaatcgcaaaaccagcaagaaaagaatgaacaagaattattggaattagataaatgggcaagtttgtggaattggtttaacataacaaattggctgtggtatataaaattattcataatgatagtaggaggcttggtaggtttaagaatagtttttgctgtactttctatagtgaatagagttaggcagggatattcaccattatcgtttcagacccacctcccaaccccgaggggacccgacaggcccgaaggaatagaagaagaaggtggagagagagacagagacagatccattcgattagtgaacggatctcgacggtatcggttaacttttaaaagaaaaggggggattggggggtacagtgcaggggaaagaatagtagacataatagcaacagacatacaaactaaagaattacaaaaacaaattacaaaaattcaaaattttatcgatcacgagactagcctcgaggcatgcctgcaggaattccgttacataacttacggtaaatggcccgcctggctgaccgcccaacgacccccgcccattgacgtcaataatgacgtatgttcccatagtaacgccaatagggactttccattgacgtcaatgggtggagtatttacggtaaactgcccacttggcagtacatcaagtgtatcatatgccaagtacgccccctattgacgtcaatgacggtaaatggcccgcctggcattatgcccagtacatgaccttatgggactttcctacttggcagtacatctacgtattagtcatcgctattaccatggtcgaggtgagccccacgttctgcttcactctccccatctcccccccctccccacccccaattttgtatttatttattttttaattattttgtgcagcgatgggggcggggggggggggggggcgcgcgccaggcggggcggggcggggcgaggggcggggcggggcgaggcggagaggtgcggcggcagccaatcagagcggcgcgctccgaaagtttccttttatggcgaggcggcggcggcggcggccctataaaaagcgaagcgcgcggcgggcgggagtcgctgcgacgctgccttcgccccgtgccccgctccgccgccgcctcgcgccgcccgccccggctctgactgaccgcgttactcccacaggtgagcgggcgggacggcccttctcctccgggctgtaattagctgagcaagaggtaagggtttaagggatggttggttggtggggtattaatgtttaattacctggagcacctgcctgaaatcactttttttcaggttggaccggtacgcgtgccaccatggatgcaatgaagagagggctctgctgtgtgctgctgctgtgtggagcagtcttcgtttcgcccagcgagctgacacaggaccctgccgtgtccgtggccctgaagcagaccgtgacaatcacctgcagaggcgattccctgagatcccactacgcctcctggtaccagaagaagcctggccaggcccccgtgctgctgttttacggcaagaataaccgccccagcggcatccccgatagattttccggcagcgcctccggcaacagagccagcctgacaatcaccggcgcccaggccgaggacgaggctgattactactgcagctccagagataagagcggcagcagactgtccgtgtttggcggcggcaccaagctgaccgtgctcggaggaggaggaagcggaggaggaggctcaggcggcggcggctctgaggtgaggctgagagagtccggcggcggcctggtgaagcccggaggatctctgaggctgtcctgctccgcctccggcttcgattttgacaatgcctggatgacctgggtgagacagccccctggcaagggcctggagtgggtgggaaggatcacaggccccggcgagggctggtccgtggattacgccgagtccgtgaagggcaggttcacaatctccagggataacaccaagaacaccctgtacctggagatgaacaacgtgaggacagaggataccggctactacttttgcgccagaacaggcaagtactacgacttttggttcggctacccccctggcgaggagtacttccaggattggggccagggcaccctggtcattgtgtccagcggcggcggcggcagtggcggcggcggaagcggcggcggcggctctggcggcggcggcagcggcggcggcggctccgacatcgtgatgacccagtctcctgatagcctggccgtgagcctgggcgagagagtgacaatgaactgtaagtctagccagagcctgctgtactccaccaaccagaagaattacctggcctggtatcagcagaagcctggccagtccccaaagctgctgatctattgggcatctacaagggagagcggagtgccagacagattcagcggatccggatctggaaccgacttcaccctgacaatctcctctgtgcaggccgaggacgtggccgtgtactattgccagcagtactatagctacaggacattcggcggcggcaccaagctggagatcaagcgcaccgtggccggaggaggaggatctggcggaggagggtccggcggcggcggctcccaggtgcagctgcagcagagcggaccagaggtggtgaagcctggagcctccgtgaagatgtcttgtaaggccagcggctacaccttcacatcctatgtgatccactgggtgaggcagaagccaggacagggactggactggatcggctacatcaacccttataatgatggcaccgactacgatgagaagtttaagggcaaggccaccctgacatccgataccagcacatccaccgcctatatggagctgagctccctgcggtctgaggacacagccgtgtactattgcgccagagagaaggataactacgcaaccggagcatggttcgcatattggggacagggtaccctggtcaccgtgtctagcgagcccaagagctgtgacaagacacacacctgccctccatgtccagcaccagagctgctgggagggccctccgtgttcctgtttccccctaagccaaaggatacactgatgatctccaggacaccagaggtgacctgcgtggtggtggacgtgtctcacgaggatcctgaggtgaagtttaactggtacgtggacggcgtggaggtgcacaatgccaagaccaagcctagggaggagcagtacaattctacatatcgcgtggtgagcgtgctgaccgtgctgcaccaggattggctgaacggcaaggagtataagtgcaaggtgagcaataaggccctgcctgccccaatcgagaagacaatctccaaggcaaagggacagccaagggagcctcaggtgtacaccctgccaccctctcgcgacgagctgacaaagaaccaggtgagcctgacctgtctggtgaagggcttctatcctagcgatattgccgtggagtgggagtccaatggccagccagagaacaattacaagaccacacctccagtgctggactccgatggctctttctttctgtattccaagctgacagtggacaagtctagatggcagcagggcaacgtgttttcttgtagcgtgatgcacgaggccctgcacaatcactacacccagaagtccctgtctctgagccccggcaagtaggatatccagcacagtcccgggccgagtctagacgtttaaacccgctgatcaggtcgacaatcaacctctggattacaaaatttgtgaaagattgactggtattcttaactatgttgctccttttacgctatgtggatacgctgctttaatgcctttgtatcatgctattgcttcccgtatggctttcattttctcctccttgtataaatcctggttgctgtctctttatgaggagttgtggcccgttgtcaggcaacgtggcgtggtgtgcactgtgtttgctgacgcaacccccactggttggggcattgccaccacctgtcagctcctttccgggactttcgctttccccctccctattgccacggcggaactcatcgccgcctgccttgcccgctgctggacaggggctcggctgttgggcactgacaattccgtggtgttgtcggggaagctgacgtcctttccatggctgctcgcctgtgttgccacctggattctgcgcgggacgtccttctgctacgtcccttcggccctcaatccagcggaccttccttcccgcggcctgctgccggctctgcggcctcttccgcgtcttcgccttcgccctcagacgagtcggatctccctttgggccgcctccccgcggtacctttaagaccaatgacttacaaggcagctgtagatcttagccactttttaaaagaaaaggggggactggaagggctaattcactcccaacgaagacaagatctgctttttgcttgtactgggtctctctggttagaccagatctgagcctgggagctctctggctaactagggaacccactgcttaagcctcaataaagcttgccttgagtgcttcaagtagtgtgtgcccgtctgttgtgtgactctggtaactagagatccctcagacccttttagtcagtgtggaaaatctctagcagtagtagttcatgtcatcttattattcagtatttataacttgcaaagaaatgaatatcagagagtgagaggaacttgtttattgcagcttataatggttacaaataaagcaatagcatcacaaatttcacaaataaagcatttttttcactgcattctagttgtggtttgtccaaactcatcaatgtatcttatcatgtctggctctagctatcccgcccctaactccgcccatcccgcccctaactccgcccagttccgcccattctccgccccatggctgactaattttttttatttatgcagaggccgaggccgcctcggcctctgagctattccagaagtagtgaggaggcttttttggaggccgctagcgtcgaccattacttattgttttagctgtcctcatgaatgtcttttcactacccatttgcttatcctgcatctctcagccttgactccactcagttctcttgcttagagataccacctttcccctgaagtgttccttccatgttttacggcgagatggtttctcctcgcctggccactcagccttagttgtctctgttgtcttatagaggtctacttgaagaaggaaaaacagggggcatggtttgactgtcctgtgagcccttcttccctgcctcccccactcacagtgacccggaatccctcgacatggcagtctagcactagtgcggccgcagatctgcttcctcgctcactgactcgctgcgctcggtcgttcggctgcggcgagcggtatcagctcactcaaaggcggtaatacggttatccacagaatcaggggataacgcaggaaagaacatgtgagcaaaaggccagcaaaaggccaggaaccgtaaaaa

SEQ ID NO: 12 - DNA, 8960 bp, Artificial Sequence
ggccgcgttgctggcgtttttccataggctccgcccccctgacgagcatcacaaaaatcgacgctcaagtcagaggtggcgaaacccgacaggactataaagataccaggcgtttccccctggaagctccctcgtgcgctctcctgttccgaccctgccgcttaccggatacctgtccgcctttctcccttcgggaagcgtggcgctttctcatagctcacgctgtaggtatctcagttcggtgtaggtcgttcgctccaagctgggctgtgtgcacgaaccccccgttcagcccgaccgctgcgccttatccggtaactatcgtcttgagtccaacccggtaagacacgacttatcgccactggcagcagccactggtaacaggattagcagagcgaggtatgtaggcggtgctacagagttcttgaagtggtggcctaactacggctacactagaagaacagtatttggtatctgcgctctgctgaagccagttaccttcggaaaaagagttggtagctcttgatccggcaaacaaaccaccgctggtagcggtggtttttttgtttgcaagcagcagattacgcgcagaaaaaaaggatctcaagaagatcctttgatcttttctacggggtctgacgctcagtggaacgaaaactcacgttaagggattttggtcatgaagcgcttttgaagctcggatccgaacaaacgacccaacacccgtgcgttttattctgtctttttattgccgatcccctcagaagaactcgtcaagaaggcgatagaaggcgatgcgctgcgaatcgggagcggcgataccgtaaagcacgaggaagcggtcagcccattcgccgccaagctcttcagcaatatcacgggtagccaacgctatgtcctgatagcggtccgccacacccagccggccacagtcgatgaatccagaaaagcggccattttccaccatgatattcggcaagcaggcatcgccatgggtcacgacgagatcctcgccgtcgggcatgctcgccttgagcctggcgaacagttcggctggcgcgagcccctgatgctcttcgtccagatcatcctgatcgacaagaccggcttccatccgagtacgtgctcgctcgatgcgatgtttcgcttggtggtcgaatgggcaggtagccggatcaagcgtatgcagccgccgcattgcatcagccatgatggatactttctcggcaggagcaaggtgagatgacaggagatcctgccccggcacttcgcccaatagcagccagtcccttcccgcttcagtgacaacgtcgagcacagctgcgcaaggaacgcccgtcgtggccagccacgatagccgcgctgcctcgtcttgcagttcattcagggcaccggacaggtcggtcttgacaaaaagaaccgggcgcccctgcgctgacagccggaacacggcggcatcagagcagccgattgtctgttgtgcccagtcatagccgaatagcctctccacccaagcggccggagaacctgcgtgcaatccatcttgttcaatcatgcgaaacgatcctcatcctgtctcttgatcagagcttgatcccctgcgccatcagatccttggcggcaagaaagccatccagtttactttgcagggcttcccaaccttaccagaggcctgcgccgcggccagctggctagcaattcccgggttaactctagagacattgattattgactagttattaatagtaatcaattacggggtcattagttcatagcccatatatggagttccgcgttacataacttacggtaaatggcccgcctggctgaccgcccaacgacccccgcccattgacgtcaataatgacgtatgttcccatagtaacgccaatagggactttccattgacgtcaatgggtggagtatttacggtaaactgcccacttggcagtacatcaagtgtatcatatgccaagtacgccccctattgacgtcaatgacggtaaatggcccgcctggcattatgcccagtacatgaccttatgggactttcctacttggcagtacatctacgtattagtcatcgctattaccatggtgatgcggttttggcagtacatcaatgggcgtggatagcggtttgactcacggggatttccaagtctccaccccattgacgtcaatgggagtttgttttggcaccaaaatcaacgggactttccaaaatgtcgtaacaactccgccccattgacgcaaatgggcggtaggcgtgtacggtgggaggtctatataagcagagctcgtttagtgaaccggggtctctctggttagaccagatctgagcctgggagctctctggctaactagggaacccactgcttaagcctcaataaagcttgccttgagtgcttcaagtagtgtgtgcccgtctgttgtgtgactctggtaactagagatccctcagacccttttagtcagtgtggaaaatctctagcagtggcgcccgaacagggacttgaaagcgaaagggaaaccagaggagctctctcgacgcaggactcggcttgctgaagcgcgcacggcaagaggcgaggggcggcgactggtgagtacgccaaaaattttgactagcggaggctagaaggagagagatgggtgcgagagcgtcagtattaagcgggggagaattagatcgcgatgggaaaaaattcggttaaggccagggggaaagaaaaaatataaattaaaacatatagtatgggcaagcagggagctagaacgattcgcagttaatcctggcctgttagaaacatcagaaggctgtagacaaatactgggacagctacaaccatcccttcagacaggatcagaagaacttagatcattatataatacagtagcaaccctctattgtgtgcatcaaaggatagagataaaagacaccaaggaagctttagacaagatagaggaagagcaaaacaaaagtaagaccaccgcacagcaagcggccgctgatcttcagacctggaggaggagatatgagggacaattggagaagtgaattatataaatataaagtagtaaaaattgaaccattaggagtagcacccaccaaggcaaagagaagagtggtgcagagagaaaaaagagcagtgggaataggagctttgttccttgggttcttgggagcagcaggaagcactatgggcgcagcgtcaatgacgctgacggtacaggccagacaattattgtctggtatagtgcagcagcagaacaatttgctgagggctattgaggcgcaacagcatctgttgcaactcacagtctggggcatcaagcagctccaggcaagaatcctggctgtggaaagatacctaaaggatcaacagctcctggggatttggggttgctctggaaaactcatttgcaccactgctgtgccttggaatgctagttggagtaataaatctctggaacagatttggaatcacacgacctggatggagtgggacagagaaattaacaattacacaagcttaatacactccttaattgaagaatcgcaaaaccagcaagaaaagaatgaacaagaattattggaattagataaatgggcaagtttgtggaattggtttaacataacaaattggctgtggtatataaaattattcataatgatagtaggaggcttggtaggtttaagaatagtttttgctgtactttctatagtgaatagagttaggcagggatattcaccattatcgtttcagacccacctcccaaccccgaggggacccgacaggcccgaaggaatagaagaagaaggtggagagagagacagagacagatccattcgattagtgaacggatctcgacggtatcggttaacttttaaaagaaaaggggggattggggggtacagtgcaggggaaagaatagtagacataatagcaacagacatacaaactaaagaattacaaaaacaaattacaaaaattcaaaattttatcgatcacgagactagcctcgaggcatgcctgcaggaattccgttacataacttacggtaaatggcccgcctggctgaccgcccaacgacccccgcccattgacgtcaataatgacgtatgttcccatagtaacgccaatagggactttccattgacgtcaatgggtggagtatttacggtaaactgcccacttggcagtacatcaagtgtatcatatgccaagtacgccccctattgacgtcaatgacggtaaatggcccgcctggcattatgcccagtacatgaccttatgggactttcctacttggcagtacatctacgtattagtcatcgctattaccatggtcgaggtgagccccacgttctgcttcactctccccatctcccccccctccccacccccaattttgtatttatttattttttaattattttgtgcagcgatgggggcggggggggggggggggcgcgcgccaggcggggcggggcggggcgaggggcggggcggggcgaggcggagaggtgcggcggcagccaatcagagcggcgcgctccgaaagtttccttttatggcgaggcggcggcggcggcggccctataaaaagcgaagcgcgcggcgggcgggagtcgctgcgacgctgccttcgccccgtgccccgctccgccgccgcctcgcgccgcccgccccggctctgactgaccgcgttactcccacaggtgagcgggcgggacggcccttctcctccgggctgtaattagctgagcaagaggtaagggtttaagggatggttggttggtggggtattaatgtttaattacctggagcacctgcctgaaatcactttttttcaggttggaccggtacgcgtgccaccatggatatgagagtgcctgcccagctgctgggcctgctgctgctgtggctgagcggcgctagatgtagcgagctgacccaggatcccgccgtgagcgtggccctgaagcagaccgtgacaatcacctgcagaggcgatagcctgagatcccactacgccagctggtaccagaagaagcctggccaggcccccgtgctgctgttctacggcaagaacaatagacctagcggcatccctgacaggttctccggcagcgcctccggcaacagggcctctctgaccatcaccggcgcccaggccgaggacgaggctgattactactgttcctccagagacaagtccggctccagactgagcgtgttcggcggcggcaccaagctgacagtgctgagccagcctaaggccgcccctagcgtgacactgttccccccttccagcgaggagctgcaggccaataaggccacactggtgtgtctgatcagcgacttttaccctggcgccgtgacagtggcctggaaggccgattccagccccgtgaaggccggcgtggagacaaccacaccctccaagcagagcaacaataagtacgccgcctcctcctacctgtccctgacccccgagcagtggaagtcccacaggtcctactcctgtcaggtgacccacgagggcagcaccgtggagaagacagtggcccccaccgagtgttccagaaagaggagagcccctgtgaagcagaccctgaatttcgatctgctgaagctggccggcgacgtggagtccaatcccggcccaatggagttcggcctgagctgggtgtttctggtggccctgttcaggggcgtgcagtgcgaggtgagactgagggagagcggcggcggcctggtgaagcctggaggaagcctgagactgtcctgtagcgccagcggctttgactttgacaatgcctggatgacctgggtgagacagcctcctggcaagggcctggagtgggtgggcagaatcaccggccccggcgagggatggtccgtggattacgccgagagcgtgaagggcagattcactatcagcagggataatacaaagaatacactgtacctggagatgaacaacgtgaggaccgaggacaccggctactacttctgtgccaggaccggcaagtactacgatttctggttcggctacccccctggcgaggagtactttcaggactggggccagggcacactggtcattgtgagctccgcctccaccaagggcccaagcgtgttccctctggccccttccagcaagagcacctccggcggcaccgccgccctgggctgtctggtgaaggactacttccccgagcctgtgaccgtgtcctggaatagcggcgccctgacctccggcgtgcacacctttcctgccgtgctgcagagctccggcctgtacagcctgtccagcgtggtgaccgtgcctagctccagcctgggcacccagacctacatctgcaatgtgaaccacaagccatccaacaccaaggtggacaagaaggtggagcccaagtcctgcgacaagacccacacctgcccaccttgccccgcccctgagctgctgggcggccctagcgtgttcctgtttccacccaagcctaaggataccctgatgatctcccgcacccctgaggtgacctgcgtggtggtggatgtgagccacgaggacccagaggtgaagttcaattggtacgtggacggcgtggaggtgcacaacgccaagaccaagccccgggaggagcagtacaactccacctaccgggtggtgtccgtgctgaccgtgctgcaccaggactggctgaacggcaaggagtacaagtgtaaggtgtccaacaaggccctgcccgccccaatcgagaagaccatcagcaaggccaagggccagcctagagagccccaggtgtacaccctgcccccatcccgcgacgagctgaccaagaaccaggtgtccctgacctgcctggtgaagggcttctacccaagcgatatcgccgtggagtgggagagcaacggccagccagagaataactacaagaccacccctcccgtgctggacagcgacggctcctttttcctgtactccaagctgaccgtggacaagtcccggtggcagcagggcaacgtgttcagctgctccgtgatgcacgaggccctgcacaaccactacacccagaagtccctgagcctgagccccggcaagagaaagaggcgggccccatgagatatccagcacagtcccgggccgagtctagacgtttaaacccgctgatcaggtcgacaatcaacctctggattacaaaatttgtgaaagattgactggtattcttaactatgttgctccttttacgctatgtggatacgctgctttaatgcctttgtatcatgctattgcttcccgtatggctttcattttctcctccttgtataaatcctggttgctgtctctttatgaggagttgtggcccgttgtcaggcaacgtggcgtggtgtgcactgtgtttgctgacgcaacccccactggttggggcattgccaccacctgtcagctcctttccgggactttcgctttccccctccctattgccacggcggaactcatcgccgcctgccttgcccgctgctggacaggggctcggctgttgggcactgacaattccgtggtgttgtcggggaagctgacgtcctttccatggctgctcgcctgtgttgccacctggattctgcgcgggacgtccttctgctacgtcccttcggccctcaatccagcggaccttccttcccgcggcctgctgccggctctgcggcctcttccgcgtcttcgccttcgccctcagacgagtcggatctccctttgggccgcctccccgcggtacctttaagaccaatgacttacaaggcagctgtagatcttagccactttttaaaagaaaaggggggactggaagggctaattcactcccaacgaagacaagatctgctttttgcttgtactgggtctctctggttagaccagatctgagcctgggagctctctggctaactagggaacccactgcttaagcctcaataaagcttgccttgagtgcttcaagtagtgtgtgcccgtctgttgtgtgactctggtaactagagatccctcagacccttttagtcagtgtggaaaatctctagcagtagtagttcatgtcatcttattattcagtatttataacttgcaaagaaatgaatatcagagagtgagaggaacttgtttattgcagcttataatggttacaaataaagcaatagcatcacaaatttcacaaataaagcatttttttcactgcattctagttgtggtttgtccaaactcatcaatgtatcttatcatgtctggctctagctatcccgcccctaactccgcccatcccgcccctaactccgcccagttccgcccattctccgccccatggctgactaattttttttatttatgcagaggccgaggccgcctcggcctctgagctattccagaagtagtgaggaggcttttttggaggccgctagcgtcgaccattacttattgttttagctgtcctcatgaatgtcttttcactacccatttgcttatcctgcatctctcagccttgactccactcagttctcttgcttagagataccacctttcccctgaagtgttccttccatgttttacggcgagatggtttctcctcgcctggccactcagccttagttgtctctgttgtcttatagaggtctacttgaagaaggaaaaacagggggcatggtttgactgtcctgtgagcccttcttccctgcctcccccactcacagtgacccggaatccctcgacatggcagtctagcactagtgcggccgcagatctgcttcctcgctcactgactcgctgcgctcggtcgttcggctgcggcgagcggtatcagctcactcaaaggcggtaatacggttatccacagaatcaggggataacgcaggaaagaacatgtgagcaaaaggccagcaaaaggccaggaaccgtaaaaa

SEQ ID NO: 13 - DNA, 9071 bp, Artificial Sequence
ggccgcgttgctggcgtttttccataggctccgcccccctgacgagcatcacaaaaatcgacgctcaagtcagaggtggcgaaacccgacaggactataaagataccaggcgtttccccctggaagctccctcgtgcgctctcctgttccgaccctgccgcttaccggatacctgtccgcctttctcccttcgggaagcgtggcgctttctcatagctcacgctgtaggtatctcagttcggtgtaggtcgttcgctccaagctgggctgtgtgcacgaaccccccgttcagcccgaccgctgcgccttatccggtaactatcgtcttgagtccaacccggtaagacacgacttatcgccactggcagcagccactggtaacaggattagcagagcgaggtatgtaggcggtgctacagagttcttgaagtggtggcctaactacggctacactagaagaacagtatttggtatctgcgctctgctgaagccagttaccttcggaaaaagagttggtagctcttgatccggcaaacaaaccaccgctggtagcggtggtttttttgtttgcaagcagcagattacgcgcagaaaaaaaggatctcaagaagatcctttgatcttttctacggggtctgacgctcagtggaacgaaaactcacgttaagggattttggtcatgaagcgcttttgaagctcggatccgaacaaacgacccaacacccgtgcgttttattctgtctttttattgccgatcccctcagaagaactcgtcaagaaggcgatagaaggcgatgcgctgcgaatcgggagcggcgataccgtaaagcacgaggaagcggtcagcccattcgccgccaagctcttcagcaatatcacgggtagccaacgctatgtcctgatagcggtccgccacacccagccggccacagtcgatgaatccagaaaagcggccattttccaccatgatattcggcaagcaggcatcgccatgggtcacgacgagatcctcgccgtcgggcatgctcgccttgagcctggcgaacagttcggctggcgcgagcccctgatgctcttcgtccagatcatcctgatcgacaagaccggcttccatccgagtacgtgctcgctcgatgcgatgtttcgcttggtggtcgaatgggcaggtagccggatcaagcgtatgcagccgccgcattgcatcagccatgatggatactttctcggcaggagcaaggtgagatgacaggagatcctgccccggcacttcgcccaatagcagccagtcccttcccgcttcagtgacaacgtcgagcacagctgcgcaaggaacgcccgtcgtggccagccacgatagccgcgctgcctcgtcttgcagttcattcagggcaccggacaggtcggtcttgacaaaaagaaccgggcgcccctgcgctgacagccggaacacggcggcatcagagcagccgattgtctgttgtgcccagtcatagccgaatagcctctccacccaagcggccggagaacctgcgtgcaatccatcttgttcaatcatgcgaaacgatcctcatcctgtctcttgatcagagcttgatcccctgcgccatcagatccttggcggcaagaaagccatccagtttactttgcagggcttcccaaccttaccagaggcctgcgccgcggccagctggctagcaattcccgggttaactctagagacattgattattgactagttattaatagtaatcaattacggggtcattagttcatagcccatatatggagttccgcgttacataacttacggtaaatggcccgcctggctgaccgcccaacgacccccgcccattgacgtcaataatgacgtatgttcccatagtaacgccaatagggactttccattgacgtcaatgggtggagtatttacggtaaactgcccacttggcagtacatcaagtgtatcatatgccaagtacgccccctattgacgtcaatgacggtaaatggcccgcctggcattatgcccagtacatgaccttatgggactttcctacttggcagtacatctacgtattagtcatcgctattaccatggtgatgcggttttggcagtacatcaatgggcgtggatagcggtttgactcacggggatttccaagtctccaccccattgacgtcaatgggagtttgttttggcaccaaaatcaacgggactttccaaaatgtcgtaacaactccgccccattgacgcaaatgggcggtaggcgtgtacggtgggaggtctatataagcagagctcgtttagtgaaccggggtctctctggttagaccagatctgagcctgggagctctctggctaactagggaacccactgcttaagcctcaataaagcttgccttgagtgcttcaagtagtgtgtgcccgtctgttgtgtgactctggtaactagagatccctcagacccttttagtcagtgtggaaaatctctagcagtggcgcccgaacagggacttgaaagcgaaagggaaaccagaggagctctctcgacgcaggactcggcttgctgaagcgcgcacggcaagaggcgaggggcggcgactggtgagtacgccaaaaattttgactagcggaggctagaaggagagagatgggtgcgagagcgtcagtattaagcgggggagaattagatcgcgatgggaaaaaattcggttaaggccagggggaaagaaaaaatataaattaaaacatatagtatgggcaagcagggagctagaacgattcgcagttaatcctggcctgttagaaacatcagaaggctgtagacaaatactgggacagctacaaccatcccttcagacaggatcagaagaacttagatcattatataatacagtagcaaccctctattgtgtgcatcaaaggatagagataaaagacaccaaggaagctttagacaagatagaggaagagcaaaacaaaagtaagaccaccgcacagcaagcggccgctgatcttcagacctggaggaggagatatgagggacaattggagaagtgaattatataaatataaagtagtaaaaattgaaccattaggagtagcacccaccaaggcaaagagaagagtggtgcagagagaaaaaagagcagtgggaataggagctttgttccttgggttcttgggagcagcaggaagcactatgggcgcagcgtcaatgacgctgacggtacaggccagacaattattgtctggtatagtgcagcagcagaacaatttgctgagggctattgaggcgcaacagcatctgttgcaactcacagtctggggcatcaagcagctccaggcaagaatcctggctgtggaaagatacctaaaggatcaacagctcctggggatttggggttgctctggaaaactcatttgcaccactgctgtgccttggaatgctagttggagtaataaatctctggaacagatttggaatcacacgacctggatggagtgggacagagaaattaacaattacacaagcttaatacactccttaattgaagaatcgcaaaaccagcaagaaaagaatgaacaagaattattggaattagataaatgggcaagtttgtggaattggtttaacataacaaattggctgtggtatataaaattattcataatgatagtaggaggcttggtaggtttaagaatagtttttgctgtactttctatagtgaatagagttaggcagggatattcaccattatcgtttcagacccacctcccaaccccgaggggacccgacaggcccgaaggaatagaagaagaaggtggagagagagacagagacagatccattcgattagtgaacggatctcgacggtatcggttaacttttaaaagaaaaggggggattggggggtacagtgcaggggaaagaatagtagacataatagcaacagacatacaaactaaagaattacaaaaacaaattacaaaaattcaaaattttatcgatcacgagactagcctcgaggcatgcctgcaggaattccgttacataacttacggtaaatggcccgcctggctgaccgcccaacgacccccgcccattgacgtcaataatgacgtatgttcccatagtaacgccaatagggactttccattgacgtcaatgggtggagtatttacggtaaactgcccacttggcagtacatcaagtgtatcatatgccaagtacgccccctattgacgtcaatgacggtaaatggcccgcctggcattatgcccagtacatgaccttatgggactttcctacttggcagtacatctacgtattagtcatcgctattaccatggtcgaggtgagccccacgttctgcttcactctccccatctcccccccctccccacccccaattttgtatttatttattttttaattattttgtgcagcgatgggggcggggggggggggggggcgcgcgccaggcggggcggggcggggcgaggggcggggcggggcgaggcggagaggtgcggcggcagccaatcagagcggcgcgctccgaaagtttccttttatggcgaggcggcggcggcggcggccctataaaaagcgaagcgcgcggcgggcgggagtcgctgcgacgctgccttcgccccgtgccccgctccgccgccgcctcgcgccgcccgccccggctctgactgaccgcgttactcccacaggtgagcgggcgggacggcccttctcctccgggctgtaattagctgagcaagaggtaagggtttaagggatggttggttggtggggtattaatgtttaattacctggagcacctgcctgaaatcactttttttcaggttggaccggtacgcgtgccaccatggatgcaatgaagagagggctctgctgtgtgctgctgctgtgtggagcagtcttcgtttcgccccagagcgccctgacacagccaccttccgcctctggaagcccaggacagagcatcaccatctcctgtaccggcacatccaacaatttcgtgtcttggtatcagcagcacgcaggcaaggcaccaaagctggtcatctacgacgtgaacaagcggccaagcggcgtgcccgatagattttccggctctaagagcggcaatacagcctctctgaccgtgagcggcctgcagaccgacgatgaggccgtgtactattgcggctccctggtgggcaactgggacgtgatcttcggcggcggcacaaagctgaccgtgctgggaggaggaggaagcggaggaggaggctcaggcggcggcggctctcagccacagctgcaggagagcggacccacactggtggaggcatccgagacactgtctctgacctgcgccgtgtccggcgattctaccgcagcctgtaatagcttttggggatgggtgcggcagccaccaggcaagggcctggagtgggtgggctccctgtctcactgcgcctcctactggaaccggggctggacctatcacaatccaagcctgaagtccagactgacactggccctggacacccccaagaacctggtgttcctgaagctgaatagcgtgacagccgccgataccgccacatactattgtgccaggtttggaggagaggtgctgaggtacaccgactggcccaagcctgcatgggtggatctgtggggaaggggcacactggtgaccgtgagctccggcggcggcggcagtggcggcggcggaagcggcggcggcggctctggcggcggcggcagcggcggcggcggctccgacatcgtgatgacccagtctcctgatagcctggccgtgagcctgggcgagagagtgacaatgaactgtaagtctagccagagcctgctgtactccaccaaccagaagaattacctggcctggtatcagcagaagcctggccagtccccaaagctgctgatctattgggcatctacaagggagagcggagtgccagacagattcagcggatccggatctggaaccgacttcaccctgacaatctcctctgtgcaggccgaggacgtggccgtgtactattgccagcagtactatagctacaggacattcggcggcggcaccaagctggagatcaagcgcaccgtggccggaggaggaggatctggcggaggagggtccggcggcggcggctcccaggtgcagctgcagcagagcggaccagaggtggtgaagcctggagcctccgtgaagatgtcttgtaaggccagcggctacaccttcacatcctatgtgatccactgggtgaggcagaagccaggacagggactggactggatcggctacatcaacccttataatgatggcaccgactacgatgagaagtttaagggcaaggccaccctgacatccgataccagcacatccaccgcctatatggagctgagctccctgcggtctgaggacacagccgtgtactattgcgccagagagaaggataactacgcaaccggagcatggttcgcatattggggacagggtaccctggtcaccgtgtctagcgagcccaagagctgtgacaagacacacacctgccctccatgtccagcaccagagctgctgggagggccctccgtgttcctgtttccccctaagccaaaggatacactgatgatctccaggacaccagaggtgacctgcgtggtggtggacgtgtctcacgaggatcctgaggtgaagtttaactggtacgtggacggcgtggaggtgcacaatgccaagaccaagcctagggaggagcagtacaattctacatatcgcgtggtgagcgtgctgaccgtgctgcaccaggattggctgaacggcaaggagtataagtgcaaggtgagcaataaggccctgcctgccccaatcgagaagacaatctccaaggcaaagggacagccaagggagcctcaggtgtacaccctgccaccctctcgcgacgagctgacaaagaaccaggtgagcctgacctgtctggtgaagggcttctatcctagcgatattgccgtggagtgggagtccaatggccagccagagaacaattacaagaccacacctccagtgctggactccgatggctctttctttctgtattccaagctgacagtggacaagtctagatggcagcagggcaacgtgttttcttgtagcgtgatgcacgaggccctgcacaatcactacacccagaagtccctgtctctgagccccggcaagtaggatatccagcacagtcccgggccgagtctagacgtttaaacccgctgatcaggtcgacaatcaacctctggattacaaaatttgtgaaagattgactggtattcttaactatgttgctccttttacgctatgtggatacgctgctttaatgcctttgtatcatgctattgcttcccgtatggctttcattttctcctccttgtataaatcctggttgctgtctctttatgaggagttgtggcccgttgtcaggcaacgtggcgtggtgtgcactgtgtttgctgacgcaacccccactggttggggcattgccaccacctgtcagctcctttccgggactttcgctttccccctccctattgccacggcggaactcatcgccgcctgccttgcccgctgctggacaggggctcggctgttgggcactgacaattccgtggtgttgtcggggaagctgacgtcctttccatggctgctcgcctgtgttgccacctggattctgcgcgggacgtccttctgctacgtcccttcggccctcaatccagcggaccttccttcccgcggcctgctgccggctctgcggcctcttccgcgtcttcgccttcgccctcagacgagtcggatctccctttgggccgcctccccgcggtacctttaagaccaatgacttacaaggcagctgtagatcttagccactttttaaaagaaaaggggggactggaagggctaattcactcccaacgaagacaagatctgctttttgcttgtactgggtctctctggttagaccagatctgagcctgggagctctctggctaactagggaacccactgcttaagcctcaataaagcttgccttgagtgcttcaagtagtgtgtgcccgtctgttgtgtgactctggtaactagagatccctcagacccttttagtcagtgtggaaaatctctagcagtagtagttcatgtcatcttattattcagtatttataacttgcaaagaaatgaatatcagagagtgagaggaacttgtttattgcagcttataatggttacaaataaagcaatagcatcacaaatttcacaaataaagcatttttttcactgcattctagttgtggtttgtccaaactcatcaatgtatcttatcatgtctggctctagctatcccgcccctaactccgcccatcccgcccctaactccgcccagttccgcccattctccgccccatggctgactaattttttttatttatgcagaggccgaggccgcctcggcctctgagctattccagaagtagtgaggaggcttttttggaggccgctagcgtcgaccattacttattgttttagctgtcctcatgaatgtcttttcactacccatttgcttatcctgcatctctcagccttgactccactcagttctcttgcttagagataccacctttcccctgaagtgttccttccatgttttacggcgagatggtttctcctcgcctggccactcagccttagttgtctctgttgtcttatagaggtctacttgaagaaggaaaaacagggggcatggtttgactgtcctgtgagcccttcttccctgcctcccccactcacagtgacccggaatccctcgacatggcagtctagcactagtgcggccgcagatctgcttcctcgctcactgactcgctgcgctcggtcgttcggctgcggcgagcggtatcagctcactcaaaggcggtaatacggttatccacagaatcaggggataacgcaggaaagaacatgtgagcaaaaggccagcaaaaggccaggaaccgtaaaaa

SEQ ID NO: 14 - DNA, 8963 bp, Artificial Sequence
ggccgcgttgctggcgtttttccataggctccgcccccctgacgagcatcacaaaaatcgacgctcaagtcagaggtggcgaaacccgacaggactataaagataccaggcgtttccccctggaagctccctcgtgcgctctcctgttccgaccctgccgcttaccggatacctgtccgcctttctcccttcgggaagcgtggcgctttctcatagctcacgctgtaggtatctcagttcggtgtaggtcgttcgctccaagctgggctgtgtgcacgaaccccccgttcagcccgaccgctgcgccttatccggtaactatcgtcttgagtccaacccggtaagacacgacttatcgccactggcagcagccactggtaacaggattagcagagcgaggtatgtaggcggtgctacagagttcttgaagtggtggcctaactacggctacactagaagaacagtatttggtatctgcgctctgctgaagccagttaccttcggaaaaagagttggtagctcttgatccggcaaacaaaccaccgctggtagcggtggtttttttgtttgcaagcagcagattacgcgcagaaaaaaaggatctcaagaagatcctttgatcttttctacggggtctgacgctcagtggaacgaaaactcacgttaagggattttggtcatgaagcgcttttgaagctcggatccgaacaaacgacccaacacccgtgcgttttattctgtctttttattgccgatcccctcagaagaactcgtcaagaaggcgatagaaggcgatgcgctgcgaatcgggagcggcgataccgtaaagcacgaggaagcggtcagcccattcgccgccaagctcttcagcaatatcacgggtagccaacgctatgtcctgatagcggtccgccacacccagccggccacagtcgatgaatccagaaaagcggccattttccaccatgatattcggcaagcaggcatcgccatgggtcacgacgagatcctcgccgtcgggcatgctcgccttgagcctggcgaacagttcggctggcgcgagcccctgatgctcttcgtccagatcatcctgatcgacaagaccggcttccatccgagtacgtgctcgctcgatgcgatgtttcgcttggtggtcgaatgggcaggtagccggatcaagcgtatgcagccgccgcattgcatcagccatgatggatactttctcggcaggagcaaggtgagatgacaggagatcctgccccggcacttcgcccaatagcagccagtcccttcccgcttcagtgacaacgtcgagcacagctgcgcaaggaacgcccgtcgtggccagccacgatagccgcgctgcctcgtcttgcagttcattcagggcaccggacaggtcggtcttgacaaaaagaaccgggcgcccctgcgctgacagccggaacacggcggcatcagagcagccgattgtctgttgtgcccagtcatagccgaatagcctctccacccaagcggccggagaacctgcgtgcaatccatcttgttcaatcatgcgaaacgatcctcatcctgtctcttgatcagagcttgatcccctgcgccatcagatccttggcggcaagaaagccatccagtttactttgcagggcttcccaaccttaccagaggcctgcgccgcggccagctggctagcaattcccgggttaactctagagacattgattattgactagttattaatagtaatcaattacggggtcattagttcatagcccatatatggagttccgcgttacataacttacggtaaatggcccgcctggctgaccgcccaacgacccccgcccattgacgtcaataatgacgtatgttcccatagtaacgccaatagggactttccattgacgtcaatgggtggagtatttacggtaaactgcccacttggcagtacatcaagtgtatcatatgccaagtacgccccctattgacgtcaatgacggtaaatggcccgcctggcattatgcccagtacatgaccttatgggactttcctacttggcagtacatctacgtattagtcatcgctattaccatggtgatgcggttttggcagtacatcaatgggcgtggatagcggtttgactcacggggatttccaagtctccaccccattgacgtcaatgggagtttgttttggcaccaaaatcaacgggactttccaaaatgtcgtaacaactccgccccattgacgcaaatgggcggtaggcgtgtacggtgggaggtctatataagcagagctcgtttagtgaaccggggtctctctggttagaccagatctgagcctgggagctctctggctaactagggaacccactgcttaagcctcaataaagcttgccttgagtgcttcaagtagtgtgtgcccgtctgttgtgtgactctggtaactagagatccctcagacccttttagtcagtgtggaaaatctctagcagtggcgcccgaacagggacttgaaagcgaaagggaaaccagaggagctctctcgacgcaggactcggcttgctgaagcgcgcacggcaagaggcgaggggcggcgactggtgagtacgccaaaaattttgactagcggaggctagaaggagagagatgggtgcgagagcgtcagtattaagcgggggagaattagatcgcgatgggaaaaaattcggttaaggccagggggaaagaaaaaatataaattaaaacatatagtatgggcaagcagggagctagaacgattcgcagttaatcctggcctgttagaaacatcagaaggctgtagacaaatactgggacagctacaaccatcccttcagacaggatcagaagaacttagatcattatataatacagtagcaaccctctattgtgtgcatcaaaggatagagataaaagacaccaaggaagctttagacaagatagaggaagagcaaaacaaaagtaagaccaccgcacagcaagcggccgctgatcttcagacctggaggaggagatatgagggacaattggagaagtgaattatataaatataaagtagtaaaaattgaaccattaggagtagcacccaccaaggcaaagagaagagtggtgcagagagaaaaaagagcagtgggaataggagctttgttccttgggttcttgggagcagcaggaagcactatgggcgcagcgtcaatgacgctgacggtacaggccagacaattattgtctggtatagtgcagcagcagaacaatttgctgagggctattgaggcgcaacagcatctgttgcaactcacagtctggggcatcaagcagctccaggcaagaatcctggctgtggaaagatacctaaaggatcaacagctcctggggatttggggttgctctggaaaactcatttgcaccactgctgtgccttggaatgctagttggagtaataaatctctggaacagatttggaatcacacgacctggatggagtgggacagagaaattaacaattacacaagcttaatacactccttaattgaagaatcgcaaaaccagcaagaaaagaatgaacaagaattattggaattagataaatgggcaagtttgtggaattggtttaacataacaaattggctgtggtatataaaattattcataatgatagtaggaggcttggtaggtttaagaatagtttttgctgtactttctatagtgaatagagttaggcagggatattcaccattatcgtttcagacccacctcccaaccccgaggggacccgacaggcccgaaggaatagaagaagaaggtggagagagagacagagacagatccattcgattagtgaacggatctcgacggtatcggttaacttttaaaagaaaaggggggattggggggtacagtgcaggggaaagaatagtagacataatagcaacagacatacaaactaaagaattacaaaaacaaattacaaaaattcaaaattttatcgatcacgagactagcctcgaggcatgcctgcaggaattccgttacataacttacggtaaatggcccgcctggctgaccgcccaacgacccccgcccattgacgtcaataatgacgtatgttcccatagtaacgccaatagggactttccattgacgtcaatgggtggagtatttacggtaaactgcccacttggcagtacatcaagtgtatcatatgccaagtacgccccctattgacgtcaatgacggtaaatggcccgcctggcattatgcccagtacatgaccttatgggactttcctacttggcagtacatctacgtattagtcatcgctattaccatggtcgaggtgagccccacgttctgcttcactctccccatctcccccccctccccacccccaattttgtatttatttattttttaattattttgtgcagcgatgggggcggggggggggggggggcgcgcgccaggcggggcggggcggggcgaggggcggggcggggcgaggcggagaggtgcggcggcagccaatcagagcggcgcgctccgaaagtttccttttatggcgaggcggcggcggcggcggccctataaaaagcgaagcgcgcggcgggcgggagtcgctgcgacgctgccttcgccccgtgccccgctccgccgccgcctcgcgccgcccgccccggctctgactgaccgcgttactcccacaggtgagcgggcgggacggcccttctcctccgggctgtaattagctgagcaagaggtaagggtttaagggatggttggttggtggggtattaatgtttaattacctggagcacctgcctgaaatcactttttttcaggttggaccggtacgcgtgccaccatggacatgagggtgcccgcccagctgctgggcctgctgctgctgtggctgagcggcgctaggtgccagagcgccctgacccagccccctagcgcttccggaagccctggccagtccatcaccatcagctgtaccggcaccagcaacaactttgtgagctggtaccagcagcacgccggcaaggcccctaagctggtcatctatgatgtgaataagaggccttccggcgtgcccgacaggttcagcggcagcaagtccggcaataccgcctccctgacagtgtccggcctgcagaccgatgacgaggccgtgtactactgcggcagcctggtgggcaattgggacgtgatcttcggcggcggcacaaagctgacagtgctgggccagcccaaggccgccccttctgtgaccctgttcccccctagctccgaggagctgcaggccaataaggccaccctggtgtgtctgatcagcgatttctaccccggcgccgtgaccgtggcctggaaggctgacagcagccccgtgaaggccggcgtggagaccaccacaccctccaagcagagcaataacaagtacgccgcctcctcctacctgtccctgacccctgagcagtggaagagccacaggtcctacagctgccaggtgacccacgagggcagcaccgtggagaagacagtggcccccaccgagtgttccaggaagagaagagcccctgtgaagcagaccctgaacttcgatctgctgaagctggccggcgacgtggagagcaaccctggccctatggagtttggcctgtcctgggtgttcctggtggccctgtttagaggcgtgcagtgtcagcctcagctgcaggagagcggccctaccctggtggaggccagcgagaccctgtccctgacatgcgccgtgtccggcgatagcacagccgcctgcaactccttttggggctgggtgagacagccccccggcaagggactggagtgggtgggatccctgagccactgtgcctcctactggaataggggctggacctaccacaaccctagcctgaagtccagactgacactggccctggatacacccaagaacctggtgttcctgaagctgaactccgtgacagccgccgataccgccacctactactgtgccagattcggcggcgaggtgctgagatacacagactggcccaagcccgcctgggtggatctgtggggcagaggcaccctggtgacagtgagctccgcctccaccaagggcccaagcgtgttccctctggccccttccagcaagagcacctccggcggcaccgccgccctgggctgtctggtgaaggactacttccccgagcctgtgaccgtgtcctggaatagcggcgccctgacctccggcgtgcacacctttcctgccgtgctgcagagctccggcctgtacagcctgtccagcgtggtgaccgtgcctagctccagcctgggcacccagacctacatctgcaatgtgaaccacaagccatccaacaccaaggtggacaagaaggtggagcccaagtcctgcgacaagacccacacctgcccaccttgccccgcccctgagctgctgggcggccctagcgtgttcctgtttccacccaagcctaaggataccctgatgatctcccgcacccctgaggtgacctgcgtggtggtggatgtgagccacgaggacccagaggtgaagttcaattggtacgtggacggcgtggaggtgcacaacgccaagaccaagccccgggaggagcagtacaactccacctaccgggtggtgtccgtgctgaccgtgctgcaccaggactggctgaacggcaaggagtacaagtgtaaggtgtccaacaaggccctgcccgccccaatcgagaagaccatcagcaaggccaagggccagcctagagagccccaggtgtacaccctgcccccatcccgcgacgagctgaccaagaaccaggtgtccctgacctgcctggtgaagggcttctacccaagcgatatcgccgtggagtgggagagcaacggccagccagagaataactacaagaccacccctcccgtgctggacagcgacggctcctttttcctgtactccaagctgaccgtggacaagtcccggtggcagcagggcaacgtgttcagctgctccgtgatgcacgaggccctgcacaaccactacacccagaagtccctgagcctgagccccggcaagagaaagaggcgggccccatgagatatccagcacagtcccgggccgagtctagacgtttaaacccgctgatcaggtcgacaatcaacctctggattacaaaatttgtgaaagattgactggtattcttaactatgttgctccttttacgctatgtggatacgctgctttaatgcctttgtatcatgctattgcttcccgtatggctttcattttctcctccttgtataaatcctggttgctgtctctttatgaggagttgtggcccgttgtcaggcaacgtggcgtggtgtgcactgtgtttgctgacgcaacccccactggttggggcattgccaccacctgtcagctcctttccgggactttcgctttccccctccctattgccacggcggaactcatcgccgcctgccttgcccgctgctggacaggggctcggctgttgggcactgacaattccgtggtgttgtcggggaagctgacgtcctttccatggctgctcgcctgtgttgccacctggattctgcgcgggacgtccttctgctacgtcccttcggccctcaatccagcggaccttccttcccgcggcctgctgccggctctgcggcctcttccgcgtcttcgccttcgccctcagacgagtcggatctccctttgggccgcctccccgcggtacctttaagaccaatgacttacaaggcagctgtagatcttagccactttttaaaagaaaaggggggactggaagggctaattcactcccaacgaagacaagatctgctttttgcttgtactgggtctctctggttagaccagatctgagcctgggagctctctggctaactagggaacccactgcttaagcctcaataaagcttgccttgagtgcttcaagtagtgtgtgcccgtctgttgtgtgactctggtaactagagatccctcagacccttttagtcagtgtggaaaatctctagcagtagtagttcatgtcatcttattattcagtatttataacttgcaaagaaatgaatatcagagagtgagaggaacttgtttattgcagcttataatggttacaaataaagcaatagcatcacaaatttcacaaataaagcatttttttcactgcattctagttgtggtttgtccaaactcatcaatgtatcttatcatgtctggctctagctatcccgcccctaactccgcccatcccgcccctaactccgcccagttccgcccattctccgccccatggctgactaattttttttatttatgcagaggccgaggccgcctcggcctctgagctattccagaagtagtgaggaggcttttttggaggccgctagcgtcgaccattacttattgttttagctgtcctcatgaatgtcttttcactacccatttgcttatcctgcatctctcagccttgactccactcagttctcttgcttagagataccacctttcccctgaagtgttccttccatgttttacggcgagatggtttctcctcgcctggccactcagccttagttgtctctgttgtcttatagaggtctacttgaagaaggaaaaacagggggcatggtttgactgtcctgtgagcccttcttccctgcctcccccactcacagtgacccggaatccctcgacatggcagtctagcactagtgcggccgcagatctgcttcctcgctcactgactcgctgcgctcggtcgttcggctgcggcgagcggtatcagctcactcaaaggcggtaatacggttatccacagaatcaggggataacgcaggaaagaacatgtgagcaaaaggccagcaaaaggccaggaaccgtaaaaa

SEQ ID NO: 15 - DNA, 4400 bp, Artificial Sequence
acatgtgagcaaaaggccagcaaaaggccaggaaccgtaaaaaggccgcgttgctggcgtttttccataggctccgcccccctgacgagcatcacaaaaatcgacgctcaagtcagaggtggcgaaacccgacaggactataaagataccaggcgtttccccctggaagctccctcgtgcgctctcctgttccgaccctgccgcttaccggatacctgtccgcctttctcccttcgggaagcgtggcgctttctcatagctcacgctgtaggtatctcagttcggtgtaggtcgttcgctccaagctgggctgtgtgcacgaaccccccgttcagcccgaccgctgcgccttatccggtaactatcgtcttgagtccaacccggtaagacacgacttatcgccactggcagcagccactggtaacaggattagcagagcgaggtatgtaggcggtgctacagagttcttgaagtggtggcctaactacggctacactagaaggacagtatttggtatctgcgctctgctgaagccagttaccttcggaaaaagagttggtagctcttgatccggcaaacaaaccaccgctggtagcggtggtttttttgtttgcaagcagcagattacgcgcagaaaaaaaggatctcaagaagatcctttgatcttttctacggggtctgacgctcagtggaacgaaaactcacgttaagggattttggtcatgagattatcaaaaaggatcttcacctagatccttttaaattaaaaatgaagttttaaatcaatctaaagtatatatgagtaaacttggtctgacagttaccaatgcttaatcagtgaggcacctatctcagcgatctgtctatttcgttcatccatagttgcctgactccccgtcgtgtagataactacgatacgggagggcttaccatctggccccagtgctgcaatgataccgcgagacccacgctcaccggctccagatttatcagcaataaaccagccagccggaagggccgagcgcagaagtggtcctgcaactttatccgcctccatccagtctattaattgttgccgggaagctagagtaagtagttcgccagttaatagtttgcgcaacgttgttgccattgctacaggcatcgtggtgtcacgctcgtcgtttggtatggcttcattcagctccggttcccaacgatcaaggcgagttacatgatcccccatgttgtgcaaaaaagcggttagctccttcggtcctccgatcgttgtcagaagtaagttggccgcagtgttatcactcatggttatggcagcactgcataattctcttactgtcatgccatccgtaagatgcttttctgtgactggtgagtactcaaccaagtcattctgagaatagtgtatgcggcgaccgagttgctcttgcccggcgtcaatacgggataataccgcgccacatagcagaactttaaaagtgctcatcattggaaaacgttcttcggggcgaaaactctcaaggatcttaccgctgttgagatccagttcgatgtaacccactcgtgcacccaactgatcttcagcatcttttactttcaccagcgtttctgggtgagcaaaaacaggaaggcaaaatgccgcaaaaaagggaataagggcgacacggaaatgttgaatactcatactcttcctttttcaatattattgaagcatttatcagggttattgtctcatgagcggatacatatttgaatgtatttagaaaaataaacaaataggggttccgcgcacatttccccgaaaagtgccacctgacgtctaagaaaccattattatcatgacattaacctataaaaataggcgtatcacgaggccctttcgtctcgcgcgtttcggtgatgacggtgaaaacctctgacacatgcagctcccggagacggtcacagcttgtctgtaagcggatgccgggagcagacaagcccgtcagggcgcgtcagcgggtgttggcgggtgtcggggctggcttaactatgcggcatcagagcagattgtactgagagtgcaccataaaattgtaaacgttaatattttgttaaaattcgcgttaaatttttgttaaatcagctcattttttaaccaataggccgaaatcggcaaaatcccttataaatcaaaagaatagcccgagatagggttgagtgttgttccagtttggaacaagagtccactattaaagaacgtggactccaacgtcaaagggcgaaaaaccgtctatcagggcgatggcccactacgtgaaccatcacccaaatcaagttttttggggtcgaggtgccgtaaagcactaaatcggaaccctaaagggagcccccgatttagagcttgacggggaaagccggcgaacgtggcgagaaaggaagggaagaaagcgaaaggagcgggcgctagggcgctggcaagtgtagcggtcacgctgcgcgtaaccaccacacccgccgcgcttaatgcgccgctacagggcgcgtactatggttgctttgacgtatgcggtgtgaaataccgcacagatgcgtaaggagaaaataccgcatcaggcgcccctgcaggcagctgcgcgctcgctcgctcactgaggccgcccgggcaaagcccgggcgtcgggcgacctttggtcgcccggcctcagtgagcgagcgagcgcgcagagagggagtggccaactccatcactaggggttcctacgcgttagttattaatagtaatcaattacggggtcattagttcatagcccatatatggagttccgcgttacataacttacggtaaatggcccgcctggctgaccgcccaacgacccccgcccattgacgtcaataatgacgtatgttcccatagtaacgccaatagggactttccattgacgtcaatgggtggagtatttacggtaaactgcccacttggcagtacatcaagtgtatcatatgccaagtacgccccctattgacgtcaatgacggtaaatggcccgcctggcattatgcccagtacatgaccttatgggactttcctacttggcagtacatctacgtattagtcatcgctattaccatggtgatgcggttttggcagtacatcaatgggcgtggatagcggtttgactcacggggatttccaagtctccaccccattgacgtcaatgggagtttgttttggcaccaaaatcaacgggactttccaaaatgtcgtaacaactccgccccattgacgcaaatgggcggtaggcgtgtacggtgggaggtctatataagcagagctggtttagtgaaccgtcagatccgctagcgctaccggtcgccaccatggtgagcaagggcgaggagctgttcaccggggtggtgcccatcctggtcgagctggacggcgacgtaaacggccacaagttcagcgtgtccggcgagggcgagggcgatgccacctacggcaagctgaccctgaagttcatctgcaccaccggcaagctgcccgtgccctggcccaccctcgtgaccaccctgacctacggcgtgcagtgcttcagccgctaccccgaccacatgaagcagcacgacttcttcaagtccgccatgcccgaaggctacgtccaggagcgcaccatcttcttcaaggacgacggcaactacaagacccgcgccgaggtgaagttcgagggcgacaccctggtgaaccgcatcgagctgaagggcatcgacttcaaggaggacggcaacatcctggggcacaagctggagtacaactacaacagccacaacgtctatatcatggccgacaagcagaagaacggcatcaaggtgaacttcaagatccgccacaacatcgaggacggcagcgtgcagctcgccgaccactaccagcagaacacccccatcggcgacggccccgtgctgctgcccgacaaccactacctgagcacccagtccgccctgagcaaagaccccaacgagaagcgcgatcacatggtcctgctggagttcgtgaccgccgccgggatcactctcggcatggacgagctgtacaagtaggtcgacgtttatttgtgaaatttgtgatgctattgctttatttgtaaccatctagctttatttgtgaaatttgtgatgctattgctttatttgtaaccattataagctgcaataaacaagttaacaacaacaattgcattcattttatgtttcaggttcagggggagatgtgggaggttttttaaagtttaaacaggaacccctagtgatggagttggccactccctctctgcgcgctcgctcgctcactgaggccgggcgaccaaaggtcgcccgacgcccgggcggcctcagtgagcgagcgagcgcgcagctgcctgcagg

SEQ ID NO: 16 - protein, 6256 aa, Artificial Sequence
ACATGTGAGCAAAAGGCCAGCAAAAGGCCAGGAACCGTAAAAAGGCCGCGTTGCTGGCGTTTTTCCATAGGCTCCGCCCCCCTGACGAGCATCACAAAAATCGACGCTCAAGTCAGAGGTGGCGAAACCCGACAGGACTATAAAGATACCAGGCGTTTCCCCCTGGAAGCTCCCTCGTGCGCTCTCCTGTTCCGACCCTGCCGCTTACCGGATACCTGTCCGCCTTTCTCCCTTCGGGAAGCGTGGCGCTTTCTCATAGCTCACGCTGTAGGTATCTCAGTTCGGTGTAGGTCGTTCGCTCCAAGCTGGGCTGTGTGCACGAACCCCCCGTTCAGCCCGACCGCTGCGCCTTATCCGGTAACTATCGTCTTGAGTCCAACCCGGTAAGACACGACTTATCGCCACTGGCAGCAGCCACTGGTAACAGGATTAGCAGAGCGAGGTATGTAGGCGGTGCTACAGAGTTCTTGAAGTGGTGGCCTAACTACGGCTACACTAGAAGGACAGTATTTGGTATCTGCGCTCTGCTGAAGCCAGTTACCTTCGGAAAAAGAGTTGGTAGCTCTTGATCCGGCAAACAAACCACCGCTGGTAGCGGTGGTTTTTTTGTTTGCAAGCAGCAGATTACGCGCAGAAAAAAAGGATCTCAAGAAGATCCTTTGATCTTTTCTACGGGGTCTGACGCTCAGTGGAACGAAAACTCACGTTAAGGGATTTTGGTCATGAGATTATCAAAAAGGATCTTCACCTAGATCCTTTTAAATTAAAAATGAAGTTTTAAATCAATCTAAAGTATATATGAGTAAACTTGGTCTGACAGTTACCAATGCTTAATCAGTGAGGCACCTATCTCAGCGATCTGTCTATTTCGTTCATCCATAGTTGCCTGACTCCCCGTCGTGTAGATAACTACGATACGGGAGGGCTTACCATCTGGCCCCAGTGCTGCAATGATACCGCGAGACCCACGCTCACCGGCTCCAGATTTATCAGCAATAAACCAGCCAGCCGGAAGGGCCGAGCGCAGAAGTGGTCCTGCAACTTTATCCGCCTCCATCCAGTCTATTAATTGTTGCCGGGAAGCTAGAGTAAGTAGTTCGCCAGTTAATAGTTTGCGCAACGTTGTTGCCATTGCTACAGGCATCGTGGTGTCACGCTCGTCGTTTGGTATGGCTTCATTCAGCTCCGGTTCCCAACGATCAAGGCGAGTTACATGATCCCCCATGTTGTGCAAAAAAGCGGTTAGCTCCTTCGGTCCTCCGATCGTTGTCAGAAGTAAGTTGGCCGCAGTGTTATCACTCATGGTTATGGCAGCACTGCATAATTCTCTTACTGTCATGCCATCCGTAAGATGCTTTTCTGTGACTGGTGAGTACTCAACCAAGTCATTCTGAGAATAGTGTATGCGGCGACCGAGTTGCTCTTGCCCGGCGTCAATACGGGATAATACCGCGCCACATAGCAGAACTTTAAAAGTGCTCATCATTGGAAAACGTTCTTCGGGGCGAAAACTCTCAAGGATCTTACCGCTGTTGAGATCCAGTTCGATGTAACCCACTCGTGCACCCAACTGATCTTCAGCATCTTTTACTTTCACCAGCGTTTCTGGGTGAGCAAAAACAGGAAGGCAAAATGCCGCAAAAAAGGGAATAAGGGCGACACGGAAATGTTGAATACTCATACTCTTCCTTTTTCAATATTATTGAAGCATTTATCAGGGTTATTGTCTCATGAGCGGATACATATTTGAATGTATTTAGAAAAATAAACAAATAGGGGTTCCGCGCACATTTCCCCGAAAAGTGCCACCTGACGTCTAAGAAACCATTATTATCATGACATTAACCTATAAAAATAGGCGTATCACGAGGCCCTTTCGTCTCGCGCGTTTCGGTGATGACGGTGAAAACCTCTGACACATGCAGCTCCCGGAGACGGTCACAGCTTGTCTGTAAGCGGATGCCGGGAGCAGACAAGCCCGTCAGGGCGCGTCAGCGGGTGTTGGCGGGTGTCGGGGCTGGCTTAACTATGCGGCATCAGAGCAGATTGTACTGAGAGTGCACCATAAAATTGTAAACGTTAATATTTTGTTAAAATTCGCGTTAAATTTTTGTTAAATCAGCTCATTTTTTAACCAATAGGCCGAAATCGGCAAAATCCCTTATAAATCAAAAGAATAGCCCGAGATAGGGTTGAGTGTTGTTCCAGTTTGGAACAAGAGTCCACTATTAAAGAACGTGGACTCCAACGTCAAAGGGCGAAAAACCGTCTATCAGGGCGATGGCCCACTACGTGAACCATCACCCAAATCAAGTTTTTTGGGGTCGAGGTGCCGTAAAGCACTAAATCGGAACCCTAAAGGGAGCCCCCGATTTAGAGCTTGACGGGGAAAGCCGGCGAACGTGGCGAGAAAGGAAGGGAAGAAAGCGAAAGGAGCGGGCGCTAGGGCGCTGGCAAGTGTAGCGGTCACGCTGCGCGTAACCACCACACCCGCCGCGCTTAATGCGCCGCTACAGGGCGCGTACTATGGTTGCTTTGACGTATGCGGTGTGAAATACCGCACAGATGCGTAAGGAGAAAATACCGCATCAGGCGCCCCTGCAGGCAGCTGCGCGCTCGCTCGCTCACTGAGGCCGCCCGGGCAAAGCCCGGGCGTCGGGCGACCTTTGGTCGCCCGGCCTCAGTGAGCGAGCGAGCGCGCAGAGAGGGAGTGGCCAACTCCATCACTAGGGGTTCCTACGCGTCGTTACATAACTTACGGTAAATGGCCCGCCTGGCTGACCGCCCAACGACCCCCGCCCATTGACGTCAATAATGACGTATGTTCCCATAGTAACGCCAATAGGGACTTTCCATTGACGTCAATGGGTGGAGTATTTACGGTAAACTGCCCACTTGGCAGTACATCAAGTGTATCATATGCCAAGTACGCCCCCTATTGACGTCAATGACGGTAAATGGCCCGCCTGGCATTATGCCCAGTACATGACCTTATGGGACTTTCCTACTTGGCAGTACATCTACGTATTAGTCATCGCTATTACCATGGTCGAGGTGAGCCCCACGTTCTGCTTCACTCTCCCCATCTCCCCCCCCTCCCCACCCCCAATTTTGTATTTATTTATTTTTTAATTATTTTGTGCAGCGATGGGGGCGGGGGGGGGGGGGGGGCGCGCGCCAGGCGGGGCGGGGCGGGGCGAGGGGCGGGGCGGGGCGAGGCGGAGAGGTGCGGCGGCAGCCAATCAGAGCGGCGCGCTCCGAAAGTTTCCTTTTATGGCGAGGCGGCGGCGGCGGCGGCCCTATAAAAAGCGAAGCGCGCGGCGGGCGGGAGTCGCTGCGACGCTGCCTTCGCCCCGTGCCCCGCTCCGCCGCCGCCTCGCGCCGCCCGCCCCGGCTCTGACTGACCGCGTTACTCCCACAGGTGAGCGGGCGGGACGGCCCTTCTCCTCCGGGCTGTAATTAGCTGAGCAAGAGGTAAGGGTTTAAGGGATGGTTGGTTGGTGGGGTATTAATGTTTAATTACCTGGAGCACCTGCCTGAAATCACTTTTTTTCAGGTACCGGTCGCCACCATGGATGCAATGAAGAGAGGGCTCTGCTGTGTGCTGCTGCTGTGTGGAGCAGTCTTCGTTTCGCCCAGCGAGCTGACACAGGACCCTGCCGTGTCCGTGGCCCTGAAGCAGACCGTGACAATCACCTGCAGAGGCGATTCCCTGAGATCCCACTACGCCTCCTGGTACCAGAAGAAGCCTGGCCAGGCCCCCGTGCTGCTGTTTTACGGCAAGAATAACCGCCCCAGCGGCATCCCCGATAGATTTTCCGGCAGCGCCTCCGGCAACAGAGCCAGCCTGACAATCACCGGCGCCCAGGCCGAGGACGAGGCTGATTACTACTGCAGCTCCAGAGATAAGAGCGGCAGCAGACTGTCCGTGTTTGGCGGCGGCACCAAGCTGACCGTGCTCGGAGGAGGAGGAAGCGGAGGAGGAGGCTCAGGCGGCGGCGGCTCTGAGGTGAGGCTGAGAGAGTCCGGCGGCGGCCTGGTGAAGCCCGGAGGATCTCTGAGGCTGTCCTGCTCCGCCTCCGGCTTCGATTTTGACAATGCCTGGATGACCTGGGTGAGACAGCCCCCTGGCAAGGGCCTGGAGTGGGTGGGAAGGATCACAGGCCCCGGCGAGGGCTGGTCCGTGGATTACGCCGAGTCCGTGAAGGGCAGGTTCACAATCTCCAGGGATAACACCAAGAACACCCTGTACCTGGAGATGAACAACGTGAGGACAGAGGATACCGGCTACTACTTTTGCGCCAGAACAGGCAAGTACTACGACTTTTGGTTCGGCTACCCCCCTGGCGAGGAGTACTTCCAGGATTGGGGCCAGGGCACCCTGGTCATTGTGTCCAGCGGCGGCGGCGGCAGTGGCGGCGGCGGAAGCGGCGGCGGCGGCTCTGGCGGCGGCGGCAGCGGCGGCGGCGGCTCCGACATCGTGATGACCCAGTCTCCTGATAGCCTGGCCGTGAGCCTGGGCGAGAGAGTGACAATGAACTGTAAGTCTAGCCAGAGCCTGCTGTACTCCACCAACCAGAAGAATTACCTGGCCTGGTATCAGCAGAAGCCTGGCCAGTCCCCAAAGCTGCTGATCTATTGGGCATCTACAAGGGAGAGCGGAGTGCCAGACAGATTCAGCGGATCCGGATCTGGAACCGACTTCACCCTGACAATCTCCTCTGTGCAGGCCGAGGACGTGGCCGTGTACTATTGCCAGCAGTACTATAGCTACAGGACATTCGGCGGCGGCACCAAGCTGGAGATCAAGCGCACCGTGGCCGGAGGAGGAGGATCTGGCGGAGGAGGGTCCGGCGGCGGCGGCTCCCAGGTGCAGCTGCAGCAGAGCGGACCAGAGGTGGTGAAGCCTGGAGCCTCCGTGAAGATGTCTTGTAAGGCCAGCGGCTACACCTTCACATCCTATGTGATCCACTGGGTGAGGCAGAAGCCAGGACAGGGACTGGACTGGATCGGCTACATCAACCCTTATAATGATGGCACCGACTACGATGAGAAGTTTAAGGGCAAGGCCACCCTGACATCCGATACCAGCACATCCACCGCCTATATGGAGCTGAGCTCCCTGCGGTCTGAGGACACAGCCGTGTACTATTGCGCCAGAGAGAAGGATAACTACGCAACCGGAGCATGGTTCGCATATTGGGGACAGGGTACCCTGGTCACCGTGTCTAGCGAGCCCAAGAGCTGTGACAAGACACACACCTGCCCTCCATGTCCAGCACCAGAGCTGCTGGGAGGGCCCTCCGTGTTCCTGTTTCCCCCTAAGCCAAAGGATACACTGATGATCTCCAGGACACCAGAGGTGACCTGCGTGGTGGTGGACGTGTCTCACGAGGATCCTGAGGTGAAGTTTAACTGGTACGTGGACGGCGTGGAGGTGCACAATGCCAAGACCAAGCCTAGGGAGGAGCAGTACAATTCTACATATCGCGTGGTGAGCGTGCTGACCGTGCTGCACCAGGATTGGCTGAACGGCAAGGAGTATAAGTGCAAGGTGAGCAATAAGGCCCTGCCTGCCCCAATCGAGAAGACAATCTCCAAGGCAAAGGGACAGCCAAGGGAGCCTCAGGTGTACACCCTGCCACCCTCTCGCGACGAGCTGACAAAGAACCAGGTGAGCCTGACCTGTCTGGTGAAGGGCTTCTATCCTAGCGATATTGCCGTGGAGTGGGAGTCCAATGGCCAGCCAGAGAACAATTACAAGACCACACCTCCAGTGCTGGACTCCGATGGCTCTTTCTTTCTGTATTCCAAGCTGACAGTGGACAAGTCTAGATGGCAGCAGGGCAACGTGTTTTCTTGTAGCGTGATGCACGAGGCCCTGCACAATCACTACACCCAGAAGTCCCTGTCTCTGAGCCCCGGCAAGTAGGTCGACGTTTATTTGTGAAATTTGTGATGCTATTGCTTTATTTGTAACCATCTAGCTTTATTTGTGAAATTTGTGATGCTATTGCTTTATTTGTAACCATTATAAGCTGCAATAAACAAGTTAACAACAACAATTGCATTCATTTTATGTTTCAGGTTCAGGGGGAGATGTGGGAGGTTTTTTAAAGTTTAAACAGGAACCCCTAGTGATGGAGTTGGCCACTCCCTCTCTGCGCGCTCGCTCGCTCACTGAGGCCGGGCGACCAAAGGTCGCCCGACGCCCGGGCGGCCTCAGTGAGCGAGCGAGCGCGCAGCTGCCTGCAGG

SEQ ID NO: 17 - DNA, 6261 bp, Artificial Sequence
acatgtgagcaaaaggccagcaaaaggccaggaaccgtaaaaaggccgcgttgctggcgtttttccataggctccgcccccctgacgagcatcacaaaaatcgacgctcaagtcagaggtggcgaaacccgacaggactataaagataccaggcgtttccccctggaagctccctcgtgcgctctcctgttccgaccctgccgcttaccggatacctgtccgcctttctcccttcgggaagcgtggcgctttctcatagctcacgctgtaggtatctcagttcggtgtaggtcgttcgctccaagctgggctgtgtgcacgaaccccccgttcagcccgaccgctgcgccttatccggtaactatcgtcttgagtccaacccggtaagacacgacttatcgccactggcagcagccactggtaacaggattagcagagcgaggtatgtaggcggtgctacagagttcttgaagtggtggcctaactacggctacactagaaggacagtatttggtatctgcgctctgctgaagccagttaccttcggaaaaagagttggtagctcttgatccggcaaacaaaccaccgctggtagcggtggtttttttgtttgcaagcagcagattacgcgcagaaaaaaaggatctcaagaagatcctttgatcttttctacggggtctgacgctcagtggaacgaaaactcacgttaagggattttggtcatgagattatcaaaaaggatcttcacctagatccttttaaattaaaaatgaagttttaaatcaatctaaagtatatatgagtaaacttggtctgacagttaccaatgcttaatcagtgaggcacctatctcagcgatctgtctatttcgttcatccatagttgcctgactccccgtcgtgtagataactacgatacgggagggcttaccatctggccccagtgctgcaatgataccgcgagacccacgctcaccggctccagatttatcagcaataaaccagccagccggaagggccgagcgcagaagtggtcctgcaactttatccgcctccatccagtctattaattgttgccgggaagctagagtaagtagttcgccagttaatagtttgcgcaacgttgttgccattgctacaggcatcgtggtgtcacgctcgtcgtttggtatggcttcattcagctccggttcccaacgatcaaggcgagttacatgatcccccatgttgtgcaaaaaagcggttagctccttcggtcctccgatcgttgtcagaagtaagttggccgcagtgttatcactcatggttatggcagcactgcataattctcttactgtcatgccatccgtaagatgcttttctgtgactggtgagtactcaaccaagtcattctgagaatagtgtatgcggcgaccgagttgctcttgcccggcgtcaatacgggataataccgcgccacatagcagaactttaaaagtgctcatcattggaaaacgttcttcggggcgaaaactctcaaggatcttaccgctgttgagatccagttcgatgtaacccactcgtgcacccaactgatcttcagcatcttttactttcaccagcgtttctgggtgagcaaaaacaggaaggcaaaatgccgcaaaaaagggaataagggcgacacggaaatgttgaatactcatactcttcctttttcaatattattgaagcatttatcagggttattgtctcatgagcggatacatatttgaatgtatttagaaaaataaacaaataggggttccgcgcacatttccccgaaaagtgccacctgacgtctaagaaaccattattatcatgacattaacctataaaaataggcgtatcacgaggccctttcgtctcgcgcgtttcggtgatgacggtgaaaacctctgacacatgcagctcccggagacggtcacagcttgtctgtaagcggatgccgggagcagacaagcccgtcagggcgcgtcagcgggtgttggcgggtgtcggggctggcttaactatgcggcatcagagcagattgtactgagagtgcaccataaaattgtaaacgttaatattttgttaaaattcgcgttaaatttttgttaaatcagctcattttttaaccaataggccgaaatcggcaaaatcccttataaatcaaaagaatagcccgagatagggttgagtgttgttccagtttggaacaagagtccactattaaagaacgtggactccaacgtcaaagggcgaaaaaccgtctatcagggcgatggcccactacgtgaaccatcacccaaatcaagttttttggggtcgaggtgccgtaaagcactaaatcggaaccctaaagggagcccccgatttagagcttgacggggaaagccggcgaacgtggcgagaaaggaagggaagaaagcgaaaggagcgggcgctagggcgctggcaagtgtagcggtcacgctgcgcgtaaccaccacacccgccgcgcttaatgcgccgctacagggcgcgtactatggttgctttgacgtatgcggtgtgaaataccgcacagatgcgtaaggagaaaataccgcatcaggcgcccctgcaggcagctgcgcgctcgctcgctcactgaggccgcccgggcaaagcccgggcgtcgggcgacctttggtcgcccggcctcagtgagcgagcgagcgcgcagagagggagtggccaactccatcactaggggttcctacgcgtcgttacataacttacggtaaatggcccgcctggctgaccgcccaacgacccccgcccattgacgtcaataatgacgtatgttcccatagtaacgccaatagggactttccattgacgtcaatgggtggagtatttacggtaaactgcccacttggcagtacatcaagtgtatcatatgccaagtacgccccctattgacgtcaatgacggtaaatggcccgcctggcattatgcccagtacatgaccttatgggactttcctacttggcagtacatctacgtattagtcatcgctattaccatggtcgaggtgagccccacgttctgcttcactctccccatctcccccccctccccacccccaattttgtatttatttattttttaattattttgtgcagcgatgggggcggggggggggggggggcgcgcgccaggcggggcggggcggggcgaggggcggggcggggcgaggcggagaggtgcggcggcagccaatcagagcggcgcgctccgaaagtttccttttatggcgaggcggcggcggcggcggccctataaaaagcgaagcgcgcggcgggcgggagtcgctgcgacgctgccttcgccccgtgccccgctccgccgccgcctcgcgccgcccgccccggctctgactgaccgcgttactcccacaggtgagcgggcgggacggcccttctcctccgggctgtaattagctgagcaagaggtaagggtttaagggatggttggttggtggggtattaatgtttaattacctggagcacctgcctgaaatcactttttttcaggttggaccggtgccaccatggatgcaatgaagagagggctctgctgtgtgctgctgctgtgtggagcagtcttcgtttcgccccagagcgccctgacacagccaccttccgcctctggaagcccaggacagagcatcaccatctcctgtaccggcacatccaacaatttcgtgtcttggtatcagcagcacgcaggcaaggcaccaaagctggtcatctacgacgtgaacaagcggccaagcggcgtgcccgatagattttccggctctaagagcggcaatacagcctctctgaccgtgagcggcctgcagaccgacgatgaggccgtgtactattgcggctccctggtgggcaactgggacgtgatcttcggcggcggcacaaagctgaccgtgctgggaggaggaggaagcggaggaggaggctcaggcggcggcggctctcagccacagctgcaggagagcggacccacactggtggaggcatccgagacactgtctctgacctgcgccgtgtccggcgattctaccgcagcctgtaatagcttttggggatgggtgcggcagccaccaggcaagggcctggagtgggtgggctccctgtctcactgcgcctcctactggaaccggggctggacctatcacaatccaagcctgaagtccagactgacactggccctggacacccccaagaacctggtgttcctgaagctgaatagcgtgacagccgccgataccgccacatactattgtgccaggtttggaggagaggtgctgaggtacaccgactggcccaagcctgcatgggtggatctgtggggaaggggcacactggtgaccgtgagctccggcggcggcggcagtggcggcggcggaagcggcggcggcggctctggcggcggcggcagcggcggcggcggctccgacatcgtgatgacccagtctcctgatagcctggccgtgagcctgggcgagagagtgacaatgaactgtaagtctagccagagcctgctgtactccaccaaccagaagaattacctggcctggtatcagcagaagcctggccagtccccaaagctgctgatctattgggcatctacaagggagagcggagtgccagacagattcagcggatccggatctggaaccgacttcaccctgacaatctcctctgtgcaggccgaggacgtggccgtgtactattgccagcagtactatagctacaggacattcggcggcggcaccaagctggagatcaagcgcaccgtggccggaggaggaggatctggcggaggagggtccggcggcggcggctcccaggtgcagctgcagcagagcggaccagaggtggtgaagcctggagcctccgtgaagatgtcttgtaaggccagcggctacaccttcacatcctatgtgatccactgggtgaggcagaagccaggacagggactggactggatcggctacatcaacccttataatgatggcaccgactacgatgagaagtttaagggcaaggccaccctgacatccgataccagcacatccaccgcctatatggagctgagctccctgcggtctgaggacacagccgtgtactattgcgccagagagaaggataactacgcaaccggagcatggttcgcatattggggacagggtaccctggtcaccgtgtctagcgagcccaagagctgtgacaagacacacacctgccctccatgtccagcaccagagctgctgggagggccctccgtgttcctgtttccccctaagccaaaggatacactgatgatctccaggacaccagaggtgacctgcgtggtggtggacgtgtctcacgaggatcctgaggtgaagtttaactggtacgtggacggcgtggaggtgcacaatgccaagaccaagcctagggaggagcagtacaattctacatatcgcgtggtgagcgtgctgaccgtgctgcaccaggattggctgaacggcaaggagtataagtgcaaggtgagcaataaggccctgcctgccccaatcgagaagacaatctccaaggcaaagggacagccaagggagcctcaggtgtacaccctgccaccctctcgcgacgagctgacaaagaaccaggtgagcctgacctgtctggtgaagggcttctatcctagcgatattgccgtggagtgggagtccaatggccagccagagaacaattacaagaccacacctccagtgctggactccgatggctctttctttctgtattccaagctgacagtggacaagtctagatggcagcagggcaacgtgttttcttgtagcgtgatgcacgaggccctgcacaatcactacacccagaagtccctgtctctgagccccggcaagtaggtcgacgtttatttgtgaaatttgtgatgctattgctttatttgtaaccatctagctttatttgtgaaatttgtgatgctattgctttatttgtaaccattataagctgcaataaacaagttaacaacaacaattgcattcattttatgtttcaggttcagggggagatgtgggaggttttttaaagtttaaacaggaacccctagtgatggagttggccactccctctctgcgcgctcgctcgctcactgaggccgggcgaccaaaggtcgcccgacgcccgggcggcctcagtgagcgagcgagcgcgcagctgcctgcagg

SEQ ID NO: 18 - DNA, 5612 bp, Artificial Sequence
ggccgcgttgctggcgtttttccataggctccgcccccctgacgagcatcacaaaaatcgacgctcaagtcagaggtggcgaaacccgacaggactataaagataccaggcgtttccccctggaagctccctcgtgcgctctcctgttccgaccctgccgcttaccggatacctgtccgcctttctcccttcgggaagcgtggcgctttctcatagctcacgctgtaggtatctcagttcggtgtaggtcgttcgctccaagctgggctgtgtgcacgaaccccccgttcagcccgaccgctgcgccttatccggtaactatcgtcttgagtccaacccggtaagacacgacttatcgccactggcagcagccactggtaacaggattagcagagcgaggtatgtaggcggtgctacagagttcttgaagtggtggcctaactacggctacactagaagaacagtatttggtatctgcgctctgctgaagccagttaccttcggaaaaagagttggtagctcttgatccggcaaacaaaccaccgctggtagcggtggtttttttgtttgcaagcagcagattacgcgcagaaaaaaaggatctcaagaagatcctttgatcttttctacggggtctgacgctcagtggaacgaaaactcacgttaagggattttggtcatgaagcgcttttgaagctcggatccgaacaaacgacccaacacccgtgcgttttattctgtctttttattgccgatcccctcagaagaactcgtcaagaaggcgatagaaggcgatgcgctgcgaatcgggagcggcgataccgtaaagcacgaggaagcggtcagcccattcgccgccaagctcttcagcaatatcacgggtagccaacgctatgtcctgatagcggtccgccacacccagccggccacagtcgatgaatccagaaaagcggccattttccaccatgatattcggcaagcaggcatcgccatgggtcacgacgagatcctcgccgtcgggcatgctcgccttgagcctggcgaacagttcggctggcgcgagcccctgatgctcttcgtccagatcatcctgatcgacaagaccggcttccatccgagtacgtgctcgctcgatgcgatgtttcgcttggtggtcgaatgggcaggtagccggatcaagcgtatgcagccgccgcattgcatcagccatgatggatactttctcggcaggagcaaggtgagatgacaggagatcctgccccggcacttcgcccaatagcagccagtcccttcccgcttcagtgacaacgtcgagcacagctgcgcaaggaacgcccgtcgtggccagccacgatagccgcgctgcctcgtcttgcagttcattcagggcaccggacaggtcggtcttgacaaaaagaaccgggcgcccctgcgctgacagccggaacacggcggcatcagagcagccgattgtctgttgtgcccagtcatagccgaatagcctctccacccaagcggccggagaacctgcgtgcaatccatcttgttcaatcatgcgaaacgatcctcatcctgtctcttgatcagagcttgatcccctgcgccatcagatccttggcggcaagaaagccatccagtttactttgcagggcttcccaaccttaccagaggcctgcgccgcggccagctggctagcaattcccgggttaactctagagacattgattattgactagttattaatagtaatcaattacggggtcattagttcatagcccatatatggagttccgcgttacataacttacggtaaatggcccgcctggctgaccgcccaacgacccccgcccattgacgtcaataatgacgtatgttcccatagtaacgccaatagggactttccattgacgtcaatgggtggagtatttacggtaaactgcccacttggcagtacatcaagtgtatcatatgccaagtacgccccctattgacgtcaatgacggtaaatggcccgcctggcattatgcccagtacatgaccttatgggactttcctacttggcagtacatctacgtattagtcatcgctattaccatggtgatgcggttttggcagtacatcaatgggcgtggatagcggtttgactcacggggatttccaagtctccaccccattgacgtcaatgggagtttgttttggcaccaaaatcaacgggactttccaaaatgtcgtaacaactccgccccattgacgcaaatgggcggtaggcgtgtacggtgggaggtctatataagcagagctcgtttagtgaaccgtcagatcgcctggagacgccatccacgctgttttgacctccatagaagacaccgggaccgatccagcctcccctcgaagcttacatgtggtaccgagctcggatcctgagaacttcagggtgagtctatgggacccttgatgttttctttccccttcttttctatggttaagttcatgtcataggaaggggagaagtaacagggtacacatattgaccaaatcagggtaattttgcatttgtaattttaaaaaatgctttcttcttttaatatacttttttgtttatcttatttctaatactttccctaatctctttctttcagggcaataatgatacaatgtatcatgcctctttgcaccattctaaagaataacagtgataatttctgggttaaggcaatagcaatatttctgcatataaatatttctgcatataaattgtaactgatgtaagaggtttcatattgctaatagcagctacaatccagctaccattctgcttttattttatggttgggataaggctggattattctgagtccaagctaggcccttttgctaatcatgttcatacctcttatcttcctcccacagctcctgggcaacgtgctggtctgtgtgctggcccatcactttggcaaagcacgtgagatctgaattctgacactatgaagtgccttttgtacttagcctttttattcattggggtgaattgcaagttcaccatagtttttccacacaaccaaaaaggaaactggaaaaatgttccttctaattaccattattgcccgtcaagctcagatttaaattggcataatgacttaataggcacagccttacaagtcaaaatgcccaagagtcacaaggctattcaagcagacggttggatgtgtcatgcttccaaatgggtcactacttgtgatttccgctggtatggaccgaagtatataacacattccatccgatccttcactccatctgtagaacaatgcaaggaaagcattgaacaaacgaaacaaggaacttggctgaatccaggcttccctcctcaaagttgtggatatgcaactgtgacggatgccgaagcagtgattgtccaggtgactcctcaccatgtgctggttgatgaatacacaggagaatgggttgattcacagttcatcaacggaaaatgcagcaattacatatgccccactgtccataactctacaacctggcattctgactataaggtcaaagggctatgtgattctaacctcatttccatggacatcaccttcttctcagaggacggagagctatcatccctgggaaaggagggcacagggttcagaagtaactactttgcttatgaaactggaggcaaggcctgcaaaatgcaatactgcaagcattggggagtcagactcccatcaggtgtctggttcgagatggctgataaggatctctttgctgcagccagattccctgaatgcccagaagggtcaagtatctctgctccatctcagacctcagtggatgtaagtctaattcaggacgttgagaggatcttggattattccctctgccaagaaacctggagcaaaatcagagcgggtcttccaatctctccagtggatctcagctatcttgctcctaaaaacccaggaaccggtcctgctttcaccataatcaatggtaccctaaaatactttgagaccagatacatcagagtcgatattgctgctccaatcctctcaagaatggtcggaatgatcagtggaactaccacagaaagggaactgtgggatgactgggcaccatatgaagacgtggaaattggacccaatggagttctgaggaccagttcaggatataagtttcctttatacatgattggacatggtatgttggactccgatcttcatcttagctcaaaggctcaggtgttcgaacatcctcacattcaagacgctgcttcgcaacttcctgatgatgagagtttattttttggtgatactgggctatccaaaaatccaatcgagcttgtagaaggttggttcagtagttggaaaagctctattgcctcttttttctttatcatagggttaatcattggactattcttggttctccgagttggtatccatctttgcattaaattaaagcacaccaagaaaagacagatttatacagacatagagatgaaccgacttggaaagtaactcaaatcctgcacaacagattcttcatgtttggaccaaatcaacttgtgataccatgctcaaagaggcctcaattatatttgagtttttaatttttatgaaaaaaaaaaaaaaaaacggaattcaccccaccagtgcaggctgcctatcagaaagtggtggctggtgtggctaatgccctggcccacaagtatcactaagctcgctttcttgctgtccaatttctattaaaggttcctttgttccctaagtccaactactaaactgggggatattatgaagggccttgagcatctggattctgcctaataaaaaacatttattttcattgcaatgatgtatttaaattatttctgaatattttactaaaaagggaatgtgggaggtcagtgcatttaaaacataaagaaatgaagagctagttcaaaccttgggaaaatacactatatcttaaactccatgaaagaaggtgaggctgcaaacagctaatgcacattggcaacagcccctgatgcctatgccttattcatccctcagaaaaggattcaagtagaggcttgatttggaggttaaagttttgctatgctgtattttagtcgaccattacttattgttttagctgtcctcatgaatgtcttttcactacccatttgcttatcctgcatctctcagccttgactccactcagttctcttgcttagagataccacctttcccctgaagtgttccttccatgttttacggcgagatggtttctcctcgcctggccactcagccttagttgtctctgttgtcttatagaggtctacttgaagaaggaaaaacagggggcatggtttgactgtcctgtgagcccttcttccctgcctcccccactcacagtgacccggaatccctcgacatggcagtctagcactagtgcggccgcagatctgcttcctcgctcactgactcgctgcgctcggtcgttcggctgcggcgagcggtatcagctcactcaaaggcggtaatacggttatccacagaatcaggggataacgcaggaaagaacatgtgagcaaaaggccagcaaaaggccaggaaccgtaaaaa

SEQ ID NO: 19 - DNA, 3387 bp, Artificial Sequence
ggccgcgttgctggcgtttttccataggctccgcccccctgacgagcatcacaaaaatcgacgctcaagtcagaggtggcgaaacccgacaggactataaagataccaggcgtttccccctggaagctccctcgtgcgctctcctgttccgaccctgccgcttaccggatacctgtccgcctttctcccttcgggaagcgtggcgctttctcatagctcacgctgtaggtatctcagttcggtgtaggtcgttcgctccaagctgggctgtgtgcacgaaccccccgttcagcccgaccgctgcgccttatccggtaactatcgtcttgagtccaacccggtaagacacgacttatcgccactggcagcagccactggtaacaggattagcagagcgaggtatgtaggcggtgctacagagttcttgaagtggtggcctaactacggctacactagaagaacagtatttggtatctgcgctctgctgaagccagttaccttcggaaaaagagttggtagctcttgatccggcaaacaaaccaccgctggtagcggtggtttttttgtttgcaagcagcagattacgcgcagaaaaaaaggatctcaagaagatcctttgatcttttctacggggtctgacgctcagtggaacgaaaactcacgttaagggattttggtcatgaagcgcttttgaagctcggatccgaacaaacgacccaacacccgtgcgttttattctgtctttttattgccgatcccctcagaagaactcgtcaagaaggcgatagaaggcgatgcgctgcgaatcgggagcggcgataccgtaaagcacgaggaagcggtcagcccattcgccgccaagctcttcagcaatatcacgggtagccaacgctatgtcctgatagcggtccgccacacccagccggccacagtcgatgaatccagaaaagcggccattttccaccatgatattcggcaagcaggcatcgccatgggtcacgacgagatcctcgccgtcgggcatgctcgccttgagcctggcgaacagttcggctggcgcgagcccctgatgctcttcgtccagatcatcctgatcgacaagaccggcttccatccgagtacgtgctcgctcgatgcgatgtttcgcttggtggtcgaatgggcaggtagccggatcaagcgtatgcagccgccgcattgcatcagccatgatggatactttctcggcaggagcaaggtgagatgacaggagatcctgccccggcacttcgcccaatagcagccagtcccttcccgcttcagtgacaacgtcgagcacagctgcgcaaggaacgcccgtcgtggccagccacgatagccgcgctgcctcgtcttgcagttcattcagggcaccggacaggtcggtcttgacaaaaagaaccgggcgcccctgcgctgacagccggaacacggcggcatcagagcagccgattgtctgttgtgcccagtcatagccgaatagcctctccacccaagcggccggagaacctgcgtgcaatccatcttgttcaatcatgcgaaacgatcctcatcctgtctcttgatcagagcttgatcccctgcgccatcagatccttggcggcaagaaagccatccagtttactttgcagggcttcccaaccttaccagaggcctgcgccgcggccagctggctagcaattcccgggttaactctagagaatgtagtcttatgcaatactcttgtagtcttgcaacatggtaacgatgagttagcaacatgccttacaaggagagaaaaagcaccgtgcatgccgattggtggaagtaaggtggtacgatcgtgccttattaggaaggcaacagacgggtctgacatggattggacgaaccactgaattccgcattgcagagatattgtatttaagtgcctagctcgatacaataaacgccatttgaccattcaccacattggtgtgcacctccaagctcgagctcgtttagtgaaccgtcagatcgcctggagacgccatccacgctgttttgacctccatagaagacaccgggaccgatccagcctcccctcgaagctagtcgattaggcatctcctatggcaggaagaagcggagacagcgacgaagacctcctcaaggcagtcagactcatcaagtttctctatcaaagcaacccacctcccaatcccgaggggacccgacaggcccgaaggaatagaagaagaaggtggagagagagacagagacagatccattcgattagtgaacggatccttagcacttatctgggacgatctgcggagcctgtgcctcttcagctaccaccgcttgagagacttactcttgattgtaacgaggattgtggaacttctgggacgcagggggtgggaagccctcaaatattggtggaatctcctacaatattggagtcaggagctaaagaatagtgctgttagcttgctcaatgccacagctatagcagtagctgaggggacagatagggttatagaagtagtacaagaagcttggcactggccgtcgttttacaacgtcgtgatctgagcctgggagatctctggctaactagggaacccactgcttaagcctcaataaagcttgccttgagtgcttcaagtagtgtgtgcccgtctgttgtgtgactctggtaactagagatcaggaaaaccctggcgttacccaacttaatcgccttgcagcacatccccctttcgccagctggcgtaatagcgaagaggcccgcaccgatcgcccttcccaacagttgcgcagcctgaatggcgaatggcgcctgatgcggtattttctccttacgcatctgtgcggtatttcacaccgcatacgtcaaagcaaccatagtgtcgaccattacttattgttttagctgtcctcatgaatgtcttttcactacccatttgcttatcctgcatctctcagccttgactccactcagttctcttgcttagagataccacctttcccctgaagtgttccttccatgttttacggcgagatggtttctcctcgcctggccactcagccttagttgtctctgttgtcttatagaggtctacttgaagaaggaaaaacagggggcatggtttgactgtcctgtgagcccttcttccctgcctcccccactcacagtgacccggaatccctcgacatggcagtctagcactagtgcggccgcagatctgcttcctcgctcactgactcgctgcgctcggtcgttcggctgcggcgagcggtatcagctcactcaaaggcggtaatacggttatccacagaatcaggggataacgcaggaaagaacatgtgagcaaaaggccagcaaaaggccaggaaccgtaaaaa

SEQ ID NO: 20 - DNA, 9171 bp, Artificial Sequence
ggccgcgttgctggcgtttttccataggctccgcccccctgacgagcatcacaaaaatcgacgctcaagtcagaggtggcgaaacccgacaggactataaagataccaggcgtttccccctggaagctccctcgtgcgctctcctgttccgaccctgccgcttaccggatacctgtccgcctttctcccttcgggaagcgtggcgctttctcatagctcacgctgtaggtatctcagttcggtgtaggtcgttcgctccaagctgggctgtgtgcacgaaccccccgttcagcccgaccgctgcgccttatccggtaactatcgtcttgagtccaacccggtaagacacgacttatcgccactggcagcagccactggtaacaggattagcagagcgaggtatgtaggcggtgctacagagttcttgaagtggtggcctaactacggctacactagaagaacagtatttggtatctgcgctctgctgaagccagttaccttcggaaaaagagttggtagctcttgatccggcaaacaaaccaccgctggtagcggtggtttttttgtttgcaagcagcagattacgcgcagaaaaaaaggatctcaagaagatcctttgatcttttctacggggtctgacgctcagtggaacgaaaactcacgttaagggattttggtcatgaagcgcttttgaagctcggatccgaacaaacgacccaacacccgtgcgttttattctgtctttttattgccgatcccctcagaagaactcgtcaagaaggcgatagaaggcgatgcgctgcgaatcgggagcggcgataccgtaaagcacgaggaagcggtcagcccattcgccgccaagctcttcagcaatatcacgggtagccaacgctatgtcctgatagcggtccgccacacccagccggccacagtcgatgaatccagaaaagcggccattttccaccatgatattcggcaagcaggcatcgccatgggtcacgacgagatcctcgccgtcgggcatgctcgccttgagcctggcgaacagttcggctggcgcgagcccctgatgctcttcgtccagatcatcctgatcgacaagaccggcttccatccgagtacgtgctcgctcgatgcgatgtttcgcttggtggtcgaatgggcaggtagccggatcaagcgtatgcagccgccgcattgcatcagccatgatggatactttctcggcaggagcaaggtgagatgacaggagatcctgccccggcacttcgcccaatagcagccagtcccttcccgcttcagtgacaacgtcgagcacagctgcgcaaggaacgcccgtcgtggccagccacgatagccgcgctgcctcgtcttgcagttcattcagggcaccggacaggtcggtcttgacaaaaagaaccgggcgcccctgcgctgacagccggaacacggcggcatcagagcagccgattgtctgttgtgcccagtcatagccgaatagcctctccacccaagcggccggagaacctgcgtgcaatccatcttgttcaatcatgcgaaacgatcctcatcctgtctcttgatcagagcttgatcccctgcgccatcagatccttggcggcaagaaagccatccagtttactttgcagggcttcccaaccttaccagaggcctgcgccgcggccagctggctagcaattcccgggttaactctagagacattgattattgactagttattaatagtaatcaattacggggtcattagttcatagcccatatatggagttccgcgttacataacttacggtaaatggcccgcctggctgaccgcccaacgacccccgcccattgacgtcaataatgacgtatgttcccatagtaacgccaatagggactttccattgacgtcaatgggtggagtatttacggtaaactgcccacttggcagtacatcaagtgtatcatatgccaagtacgccccctattgacgtcaatgacggtaaatggcccgcctggcattatgcccagtacatgaccttatgggactttcctacttggcagtacatctacgtattagtcatcgctattaccatggtgatgcggttttggcagtacatcaatgggcgtggatagcggtttgactcacggggatttccaagtctccaccccattgacgtcaatgggagtttgttttggcaccaaaatcaacgggactttccaaaatgtcgtaacaactccgccccattgacgcaaatgggcggtaggcgtgtacggtgggaggtctatataagcagagctcgtttagtgaaccgtcagatcgcctggagacgccatccacgctgttttgacctccatagaagacaccgggaccgatccagcctcccctcgaagcttacatgtggtaccgagctcggatcctgagaacttcagggtgagtctatgggacccttgatgttttctttccccttcttttctatggttaagttcatgtcataggaaggggagaagtaacagggtacacatattgaccaaatcagggtaattttgcatttgtaattttaaaaaatgctttcttcttttaatatacttttttgtttatcttatttctaatactttccctaatctctttctttcagggcaataatgatacaatgtatcatgcctctttgcaccattctaaagaataacagtgataatttctgggttaaggcaatagcaatatttctgcatataaatatttctgcatataaattgtaactgatgtaagaggtttcatattgctaatagcagctacaatccagctaccattctgcttttattttatggttgggataaggctggattattctgagtccaagctaggcccttttgctaatcatgttcatacctcttatcttcctcccacagctcctgggcaacgtgctggtctgtgtgctggcccatcactttggcaaagcacgtgagatctgaattcgagatctgccgccgccatgggtgcgagagcgtcagtattaagcgggggagaattagatcgatgggaaaaaattcggttaaggccagggggaaagaaaaaatataaattaaaacatatagtatgggcaagcagggagctagaacgattcgcagttaatcctggcctgttagaaacatcagaaggctgtagacaaatactgggacagctacaaccatcccttcagacaggatcagaagaacttagatcattatataatacagtagcaaccctctattgtgtgcatcaaaggatagagataaaagacaccaaggaagctttagacaagatagaggaagagcaaaacaaaagtaagaaaaaagcacagcaagcagcagctgacacaggacacagcaatcaggtcagccaaaattaccctatagtgcagaacatccaggggcaaatggtacatcaggccatatcacctagaactttaaatgcatgggtaaaagtagtagaagagaaggctttcagcccagaagtgatacccatgttttcagcattatcagaaggagccaccccacaagatttaaacaccatgctaaacacagtggggggacatcaagcagccatgcaaatgttaaaagagaccatcaatgaggaagctgcagaatgggatagagtgcatccagtgcatgcagggcctattgcaccaggccagatgagagaaccaaggggatcagacatcgctggaactactagtacccttcaggaacaaataggatggatgacacataatccacctatcccagtaggagaaatctataaaagatggataatcctgggattaaataaaatagtaagaatgtatagccctaccagcattctggacataagacaaggaccaaaggaaccctttagagactatgtagaccgattctataaaactctaagagccgagcaagcttcacaagaggtaaaaaattggatgacagaaaccttgttggtccaaaatgcgaacccagattgtaagactattttaaaagcattgggaccaggagcgacactagaagaaatgatgacagcatgtcagggagtggggggacccggccataaagcaagagttttggctgaagcaatgagccaagtaacaaatccagctaccataatgatacagaaaggcaattttaggaaccaaagaaagactgttaagtgtttcaattgtggcaaagaagggcacatagccaaaaattgcagggcccctaggaaaaagggctgttggaaatgtggaaaggaaggacaccaaatgaaagattgtactgagagacaggctaattttttagggaagatctggccttcccacaagggaaggccagggaattttcttcagagcagaccagagccaacagccccaccagaagagagcttcaggtttggggaagagacaacaactccctctcagaagcaggagccgatagacaaggaactgtatcctttagcttccctcagatcactctttggcagcgacccctcgtcacaataaagataggggggcaattaaaggaagctctattagatactggtgctgacgacacagtattagaagaaatgaatttgccaggaagatggaaaccaaaaatgatagggggaattggaggttttatcaaagtaagacagtatgatcagatactcatagaaatctgcggacataaagctataggtacagtattagtaggacctacacctgtcaacataattggaagaaatctgttgactcagattggctgcactttaaattttcccattagtcctattgagactgtaccagtaaaattaaagccaggaatggatggcccaaaagttaaacaatggccattgacagaagaaaaaataaaagcattagtagaaatttgtacagaaatggaaaaggaaggaaaaatttcaaaaattgggcctgaaaatccatacaatactccagtatttgccataaagaaaaaagacagtactaaatggagaaaattagtagatttcagagaacttaataagagaactcaagatttctgggaagttcaattaggaataccacatcctgcagggttaaaacagaaaaaatcagtaacagtactggatgtgggcgatgcatatttttcagttcccttagataaagacttcaggaagtatactgcatttaccatacctagtataaacaatgagacaccagggattagatatcagtacaatgtgcttccacagggatggaaaggatcaccagcaatattccagtgtagcatgacaaaaatcttagagccttttagaaaacaaaatccagacatagtcatctatcaatacatggatgatttgtatgtaggatctgacttagaaatagggcagcatagaacaaaaatagaggaactgagacaacatctgttgaggtggggatttaccacaccagacaaaaaacatcagaaagaacctccattcctttggatgggttatgaactccatcctgataaatggacagtacagcctatagtgctgccagaaaaggacagctggactgtcaatgacatacagaaattagtgggaaaattgaattgggcaagtcagatttatgcagggattaaagtaaggcaattatgtaaacttcttaggggaaccaaagcactaacagaagtagtaccactaacagaagaagcagagctagaactggcagaaaacagggagattctaaaagaaccggtacatggagtgtattatgacccatcaaaagacttaatagcagaaatacagaagcaggggcaaggccaatggacatatcaaatttatcaagagccatttaaaaatctgaaaacaggaaagtatgcaagaatgaagggtgcccacactaatgatgtgaaacaattaacagaggcagtacaaaaaatagccacagaaagcatagtaatatggggaaagactcctaaatttaaattacccatacaaaaggaaacatgggaagcatggtggacagagtattggcaagccacctggattcctgagtgggagtttgtcaatacccctcccttagtgaagttatggtaccagttagagaaagaacccataataggagcagaaactttctatgtagatggggcagccaatagggaaactaaattaggaaaagcaggatatgtaactgacagaggaagacaaaaagttgtccccctaacggacacaacaaatcagaagactgagttacaagcaattcatctagctttgcaggattcgggattagaagtaaacatagtgacagactcacaatatgcattgggaatcattcaagcacaaccagataagagtgaatcagagttagtcagtcaaataatagagcagttaataaaaaaggaaaaagtctacctggcatgggtaccagcacacaaaggaattggaggaaatgaacaagtagataaattggtcagtgctggaatcaggaaagtactatttttagatggaatagataaggcccaagaagaacatgagaaatatcacagtaattggagagcaatggctagtgattttaacctaccacctgtagtagcaaaagaaatagtagccagctgtgataaatgtcagctaaaaggggaagccatgcatggacaagtagactgtagcccaggaatatggcagctagattgtacacatttagaaggaaaagttatcttggtagcagttcatgtagccagtggatatatagaagcagaagtaattccagcagagacagggcaagaaacagcatacttcctcttaaaattagcaggaagatggccagtaaaaacagtacatacagacaatggcagcaatttcaccagtactacagttaaggccgcctgttggtgggcggggatcaagcaggaatttggcattccctacaatccgcagtcacaaggagtaatagaatctatgaataaagaattaaagaaaattataggacaggtaagagatcaggctgaacatcttaaaacagcagtacaaatggcagtattcatccacaattttaaaagaaaaggggggattggggggtacagtgcaggggaaagaatagtagacataatagcaacagacatacaaactaaagaattacaaaaacaaattacaaaaattcaaaattttcgggtttattacagggacagcagagatccagtttggaaaggaccagcaaagctcctctggaaaggtgaaggggcagtagtaatacaagataatagtgacataaaagtagtgccaagaagaaaagcaaagatcatcagggattatggaaaacagatggcaggtgatgattgtgtggcaagtagacaggatgaggattaacacatggaattccggagcggccgcaggagctttgttccttgggttcttgggagcagcaggaagcactatgggcgcagcgtcaatgacgctgacggtacaggccagacaattattgtctggtatagtgcagcagcagaacaatttgctgagggctattgaggcgcaacagcatctgttgcaactcacagtctggggcatcaagcagctccaggcaagaatcctggctgtggaaagatacctaaaggatcaacagctcctggggatttggggttgctctggaaaactcatttgcaccactgctgtgccttggaatgctagttggagtaataaatctctggaacagatttggaatcacacgacctggatggagtgggacagagaaattaacaattacacaagcttccgcggaattcaccccaccagtgcaggctgcctatcagaaagtggtggctggtgtggctaatgccctggcccacaagtatcactaagctcgctttcttgctgtccaatttctattaaaggttcctttgttccctaagtccaactactaaactgggggatattatgaagggccttgagcatctggattctgcctaataaaaaacatttattttcattgcaatgatgtatttaaattatttctgaatattttactaaaaagggaatgtgggaggtcagtgcatttaaaacataaagaaatgaagagctagttcaaaccttgggaaaatacactatatcttaaactccatgaaagaaggtgaggctgcaaacagctaatgcacattggcaacagcccctgatgcctatgccttattcatccctcagaaaaggattcaagtagaggcttgatttggaggttaaagttttgctatgctgtattttacattacttattgttttagctgtcctcatgaatgtcttttcactacccatttgcttatcctgcatctctcagccttgactccactcagttctcttgcttagagataccacctttcccctgaagtgttccttccatgttttacggcgagatggtttctcctcgcctggccactcagccttagttgtctctgttgtcttatagaggtctacttgaagaaggaaaaacagggggcatggtttgactgtcctgtgagcccttcttccctgcctcccccactcacagtgacccggaatccctcgacatggcagtctagcactagtgcggccgcagatctgcttcctcgctcactgactcgctgcgctcggtcgttcggctgcggcgagcggtatcagctcactcaaaggcggtaatacggttatccacagaatcaggggataacgcaggaaagaacatgtgagcaaaaggccagcaaaaggccaggaaccgtaaaaagtcgaccattacttattgttttagctgtcctcatgaatgtcttttcactacccatttgcttatcctgcatctctcagccttgactccactcagttctcttgcttagagataccacctttcccctgaagtgttccttccatgttttacggcgagatggtttctcctcgcctggccactcagccttagttgtctctgttgtcttatagaggtctacttgaagaaggaaaaacagggggcatggtttgactgtcctgtgagcccttcttccctgcctcccccactcacagtgacccggaatccctcgacatggcagtctagcactagtgcggccgcagatctgcttcctcgctcactgactcgctgcgctcggtcgttcggctgcggcgagcggtatcagctcactcaaaggcggtaatacggttatccacagaatcaggggataacgcaggaaagaacatgtgagcaaaaggccagcaaaaggccaggaaccgtaaaaa

SEQ ID NO: 21 - DNA, 7336 bp, Artificial Sequence
atgccggggttttacgagattgtgattaaggtccccagcgaccttgacgagcatctgcccggcatttctgacagctttgtgaactgggtggccgagaaggaatgggagttgccgccagattctgacatggatctgaatctgattgagcaggcacccctgaccgtggccgagaagctgcagcgcgactttctgacggaatggcgccgtgtgagtaaggccccggaggctcttttctttgtgcaatttgagaagggagagagctacttccacatgcacgtgctcgtggaaaccaccggggtgaaatccatggttttgggacgtttcctgagtcagattcgcgaaaaactgattcagagaatttaccgcgggatcgagccgactttgccaaactggttcgcggtcacaaagaccagaaatggcgccggaggcgggaacaaggtggtggatgagtgctacatccccaattacttgctccccaaaacccagcctgagctccagtgggcgtggactaatatggaacagtatttaagcgcctgtttgaatctcacggagcgtaaacggttggtggcgcagcatctgacgcacgtgtcgcagacgcaggagcagaacaaagagaatcagaatcccaattctgatgcgccggtgatcagatcaaaaacttcagccaggtacatggagctggtcgggtggctcgtggacaaggggattacctcggagaagcagtggatccaggaggaccaggcctcatacatctccttcaatgcggcctccaactcgcggtcccaaatcaaggctgccttggacaatgcgggaaagattatgagcctgactaaaaccgcccccgactacctggtgggccagcagcccgtggaggacatttccagcaatcggatttataaaattttggaactaaacgggtacgatccccaatatgcggcttccgtctttctgggatgggccacgaaaaagttcggcaagaggaacaccatctggctgtttgggcctgcaactaccgggaagaccaacatcgcggaggccatagcccacactgtgcccttctacgggtgcgtaaactggaccaatgagaactttcccttcaacgactgtgtcgacaagatggtgatctggtgggaggaggggaagatgaccgccaaggtcgtggagtcggccaaagccattctcggaggaagcaaggtgcgcgtggaccagaaatgcaagtcctcggcccagatagacccgactcccgtgatcgtcacctccaacaccaacatgtgcgccgtgattgacgggaactcaacgaccttcgaacaccagcagccgttgcaagaccggatgttcaaatttgaactcacccgccgtctggatcatgactttgggaaggtcaccaagcaggaagtcaaagactttttccggtgggcaaaggatcacgtggttgaggtggagcatgaattctacgtcaaaaagggtggagccaagaaaagacccgcccccagtgacgcagatataagtgagcccaaacgggtgcgcgagtcagttgcgcagccatcgacgtcagacgcggaagcttcgatcaactacgcagacaggtaccaaaacaaatgttctcgtcacgtgggcatgaatctgatgctgtttccctgcagacaatgcgagagaatgaatcagaattcaaatatctgcttcactcacggacagaaagactgtttagagtgctttcccgtgtcagaatctcaacccgtttctgtcgtcaaaaaggcgtatcagaaactgtgctacattcatcatatcatgggaaaggtgccagacgcttgcactgcctgcgatctggtcaatgtggatttggatgactgcatctttgaacaataaatgatttaaatcaggtatggctgccgatggttatcttccagattggctcgaggacaacctctctgagggcattcgcgagtggtgggcgctgaaacctggagccccgaagcccaaagccaaccagcaaaagcaggacgacggccggggtctggtgcttcctggctacaagtacctcggacccttcaacggactcgacaagggggagcccgtcaacgcggcggacgcagcggccctcgagcacgacaaggcctacgaccagcagctgcaggcgggtgacaatccgtacctgcggtataaccacgccgacgccgagtttcaggagcgtctgcaagaagatacgtcttttgggggcaacctcgggcgagcagtcttccaggccaagaagcgggttctcgaacctctcggtctggttgaggaaggcgctaagacggctcctggaaagaagagaccggtagagccatcaccccagcgttctccagactcctctacgggcatcggcaagaaaggccaacagcccgccagaaaaagactcaattttggtcagactggcgactcagagtcagttccagaccctcaacctctcggagaacctccagcagcgccctctggtgtgggacctaatacaatggctgcaggcggtggcgcaccaatggcagacaataacgaaggcgccgacggagtgggtagttcctcgggaaattggcattgcgattccacatggctgggcgacagagtcatcaccaccagcacccgaacctgggccctgcccacctacaacaaccacctctacaagcaaatctccaacgggacatcgggaggagccaccaacgacaacacctacttcggctacagcaccccctgggggtattttgactttaacagattccactgccacttttcaccacgtgactggcagcgactcatcaacaacaactggggattccggcccaagagactcagcttcaagctcttcaacatccaggtcaaggaggtcacgcagaatgaaggcaccaagaccatcgccaataacctcaccagcaccatccaggtgtttacggactcggagtaccagctgccgtacgttctcggctctgcccaccagggctgcctgcctccgttcccggcggacgtgttcatgattccccagtacggctacctaacactcaacaacggtagtcaggccgtgggacgctcctccttctactgcctggaatactttccttcgcagatgctgagaaccggcaacaacttccagtttacttacaccttcgaggacgtgcctttccacagcagctacgcccacagccagagcttggaccggctgatgaatcctctgattgaccagtacctgtactacttgtctcggactcaaacaacaggaggcacggcaaatacgcagactctgggcttcagccaaggtgggcctaatacaatggccaatcaggcaaagaactggctgccaggaccctgttaccgccaacaacgcgtctcaacgacaaccgggcaaaacaacaatagcaactttgcctggactgctgggaccaaataccatctgaatggaagaaattcattggctaatcctggcatcgctatggcaacacacaaagacgacgaggagcgtttttttcccagtaacgggatcctgatttttggcaaacaaaatgctgccagagacaatgcggattacagcgatgtcatgctcaccagcgaggaagaaatcaaaaccactaaccctgtggctacagaggaatacggtatcgtggcagataacttgcagcagcaaaacacggctcctcaaattggaactgtcaacagccagggggccttacccggtatggtctggcagaaccgggacgtgtacctgcagggtcccatctgggccaagattcctcacacggacggcaacttccacccgtctccgctgatgggcggctttggcctgaaacatcctccgcctcagatcctgatcaagaacacgcctgtacctgcggatcctccgaccaccttcaaccagtcaaagctgaactctttcatcacgcaatacagcaccggacaggtcagcgtggaaattgaatgggagctgcagaaggaaaacagcaagcgctggaaccccgagatccagtacacctccaactactacaaatctacaagtgtggactttgctgttaatacagaaggcgtgtactctgaaccccgccccattggcacccgttacctcacccgtaatctgtaattgcctgttaatcaataaaccggttgattcgtttcagttgaactttggtctctgcgaagggcgaattcgtttaaacctgcaggactagaggtcctgtattagaggtcacgtgagtgttttgcgacattttgcgacaccatgtggtcacgctgggtatttaagcccgagtgagcacgcagggtctccattttgaagcgggaggtttgaacgcgcagccgccaagccgaattctgcagatatccatcacactggcggccgctcgactagagcggccgccaccgcggtggagctccagcttttgttccctttagtgagggttaattgcgcgcttggcgtaatcatggtcatagctgtttcctgtgtgaaattgttatccgctcacaattccacacaacatacgagccggaagcataaagtgtaaagcctggggtgcctaatgagtgagctaactcacattaattgcgttgcgctcactgcccgctttccagtcgggaaacctgtcgtgccagctgcattaatgaatcggccaacgcgcggggagaggcggtttgcgtattgggcgctcttccgcttcctcgctcactgactcgctgcgctcggtcgttcggctgcggcgagcggtatcagctcactcaaaggcggtaatacggttatccacagaatcaggggataacgcaggaaagaacatgtgagcaaaaggccagcaaaaggccaggaaccgtaaaaaggccgcgttgctggcgtttttccataggctccgcccccctgacgagcatcacaaaaatcgacgctcaagtcagaggtggcgaaacccgacaggactataaagataccaggcgtttccccctggaagctccctcgtgcgctctcctgttccgaccctgccgcttaccggatacctgtccgcctttctcccttcgggaagcgtggcgctttctcatagctcacgctgtaggtatctcagttcggtgtaggtcgttcgctccaagctgggctgtgtgcacgaaccccccgttcagcccgaccgctgcgccttatccggtaactatcgtcttgagtccaacccggtaagacacgacttatcgccactggcagcagccactggtaacaggattagcagagcgaggtatgtaggcggtgctacagagttcttgaagtggtggcctaactacggctacactagaagaacagtatttggtatctgcgctctgctgaagccagttaccttcggaaaaagagttggtagctcttgatccggcaaacaaaccaccgctggtagcggtggtttttttgtttgcaagcagcagattacgcgcagaaaaaaaggatctcaagaagatcctttgatcttttctacggggtctgacgctcagtggaacgaaaactcacgttaagggattttggtcatgagattatcaaaaaggatcttcacctagatccttttaaattaaaaatgaagttttaaatcaatctaaagtatatatgagtaaacttggtctgacagttaccaatgcttaatcagtgaggcacctatctcagcgatctgtctatttcgttcatccatagttgcctgactccccgtcgtgtagataactacgatacgggagggcttaccatctggccccagtgctgcaatgataccgcgagacccacgctcaccggctccagatttatcagcaataaaccagccagccggaagggccgagcgcagaagtggtcctgcaactttatccgcctccatccagtctattaattgttgccgggaagctagagtaagtagttcgccagttaatagtttgcgcaacgttgttgccattgctacaggcatcgtggtgtcacgctcgtcgtttggtatggcttcattcagctccggttcccaacgatcaaggcgagttacatgatcccccatgttgtgcaaaaaagcggttagctccttcggtcctccgatcgttgtcagaagtaagttggccgcagtgttatcactcatggttatggcagcactgcataattctcttactgtcatgccatccgtaagatgcttttctgtgactggtgagtactcaaccaagtcattctgagaatagtgtatgcggcgaccgagttgctcttgcccggcgtcaatacgggataataccgcgccacatagcagaactttaaaagtgctcatcattggaaaacgttcttcggggcgaaaactctcaaggatcttaccgctgttgagatccagttcgatgtaacccactcgtgcacccaactgatcttcagcatcttttactttcaccagcgtttctgggtgagcaaaaacaggaaggcaaaatgccgcaaaaaagggaataagggcgacacggaaatgttgaatactcatactcttcctttttcaatattattgaagcatttatcagggttattgtctcatgagcggatacatatttgaatgtatttagaaaaataaacaaataggggttccgcgcacatttccccgaaaagtgccacctaaattgtaagcgttaatattttgttaaaattcgcgttaaatttttgttaaatcagctcattttttaaccaataggccgaaatcggcaaaatcccttataaatcaaaagaatagaccgagatagggttgagtgttgttccagtttggaacaagagtccactattaaagaacgtggactccaacgtcaaagggcgaaaaaccgtctatcagggcgatggcccactacgtgaaccatcaccctaatcaagttttttggggtcgaggtgccgtaaagcactaaatcggaaccctaaagggagcccccgatttagagcttgacggggaaagccggcgaacgtggcgagaaaggaagggaagaaagcgaaaggagcgggcgctagggcgctggcaagtgtagcggtcacgctgcgcgtaaccaccacacccgccgcgcttaatgcgccgctacagggcgcgtcccattcgccattcaggctgcgcaactgttgggaagggcgatcggtgcgggcctcttcgctattacgccagctggcgaaagggggatgtgctgcaaggcgattaagttgggtaacgccagggttttcccagtcacgacgttgtaaaacgacggccagtgagcgcgcgtaatacgactcactatagggcgaattgggtaccgggccccccctcgatcgaggtcgacggtatcgggggagctcgcagggtctccattttgaagcgggaggtttgaacgcgcagccgcc

SEQ ID NO: 22 - DNA, 11635 bp, Artificial Sequence
ggtacccaactccatgcttaacagtccccaggtacagcccaccctgcgtcgcaaccaggaacagctctacagcttcctggagcgccactcgccctacttccgcagccacagtgcgcagattaggagcgccacttctttttgtcacttgaaaaacatgtaaaaataatgtactaggagacactttcaataaaggcaaatgtttttatttgtacactctcgggtgattatttaccccccacccttgccgtctgcgccgtttaaaaatcaaaggggttctgccgcgcatcgctatgcgccactggcagggacacgttgcgatactggtgtttagtgctccacttaaactcaggcacaaccatccgcggcagctcggtgaagttttcactccacaggctgcgcaccatcaccaacgcgtttagcaggtcgggcgccgatatcttgaagtcgcagttggggcctccgccctgcgcgcgcgagttgcgatacacagggttgcagcactggaacactatcagcgccgggtggtgcacgctggccagcacgctcttgtcggagatcagatccgcgtccaggtcctccgcgttgctcagggcgaacggagtcaactttggtagctgccttcccaaaaagggtgcatgcccaggctttgagttgcactcgcaccgtagtggcatcagaaggtgaccgtgcccggtctgggcgttaggatacagcgcctgcatgaaagccttgatctgcttaaaagccacctgagcctttgcgccttcagagaagaacatgccgcaagacttgccggaaaactgattggccggacaggccgcgtcatgcacgcagcaccttgcgtcggtgttggagatctgcaccacatttcggccccaccggttcttcacgatcttggccttgctagactgctccttcagcgcgcgctgcccgttttcgctcgtcacatccatttcaatcacgtgctccttatttatcataatgctcccgtgtagacacttaagctcgccttcgatctcagcgcagcggtgcagccacaacgcgcagcccgtgggctcgtggtgcttgtaggttacctctgcaaacgactgcaggtacgcctgcaggaatcgccccatcatcgtcacaaaggtcttgttgctggtgaaggtcagctgcaacccgcggtgctcctcgtttagccaggtcttgcatacggccgccagagcttccacttggtcaggcagtagcttgaagtttgcctttagatcgttatccacgtggtacttgtccatcaacgcgcgcgcagcctccatgcccttctcccacgcagacacgatcggcaggctcagcgggtttatcaccgtgctttcactttccgcttcactggactcttccttttcctcttgcgtccgcataccccgcgccactgggtcgtcttcattcagccgccgcaccgtgcgcttacctcccttgccgtgcttgattagcaccggtgggttgctgaaacccaccatttgtagcgccacatcttctctttcttcctcgctgtccacgatcacctctggggatggcgggcgctcgggcttgggagaggggcgcttctttttctttttggacgcaatggccaaatccgccgtcgaggtcgatggccgcgggctgggtgtgcgcggcaccagcgcatcttgtgacgagtcttcttcgtcctcggactcgagacgccgcctcagccgcttttttgggggcgcgcggggaggcggcggcgacggcgacggggacgacacgtcctccatggttggtggacgtcgcgccgcaccgcgtccgcgctcgggggtggtttcgcgctgctcctcttcccgactggccatttccttctcctataggcagaaaaagatcatggagtcagtcgagaaggaggacagcctaaccgccccctttgagttcgccaccaccgcctccaccgatgccgccaacgcgcctaccaccttccccgtcgaggcacccccgcttgaggaggaggaagtgattatcgagcaggacccaggttttgtaagcgaagacgacgaggatcgctcagtaccaacagaggataaaaagcaagaccaggacgacgcagaggcaaacgaggaacaagtcgggcggggggaccaaaggcatggcgactacctagatgtgggagacgacgtgctgttgaagcatctgcagcgccagtgcgccattatctgcgacgcgttgcaagagcgcagcgatgtgcccctcgccatagcggatgtcagccttgcctacgaacgccacctgttctcaccgcgcgtaccccccaaacgccaagaaaacggcacatgcgagcccaacccgcgcctcaacttctaccccgtatttgccgtgccagaggtgcttgccacctatcacatctttttccaaaactgcaagatacccctatcctgccgtgccaaccgcagccgagcggacaagcagctggccttgcggcagggcgctgtcatacctgatatcgcctcgctcgacgaagtgccaaaaatctttgagggtcttggacgcgacgagaaacgcgcggcaaacgctctgcaacaagaaaacagcgaaaatgaaagtcactgtggagtgctggtggaacttgagggtgacaacgcgcgcctagccgtgctgaaacgcagcatcgaggtcacccactttgcctacccggcacttaacctaccccccaaggttatgagcacagtcatgagcgagctgatcgtgcgccgtgcacgacccctggagagggatgcaaacttgcaagaacaaaccgaggagggcctacccgcagttggcgatgagcagctggcgcgctggcttgagacgcgcgagcctgccgacttggaggagcgacgcaagctaatgatggccgcagtgcttgttaccgtggagcttgagtgcatgcagcggttctttgctgacccggagatgcagcgcaagctagaggaaacgttgcactacacctttcgccagggctacgtgcgccaggcctgcaaaatttccaacgtggagctctgcaacctggtctcctaccttggaattttgcacgaaaaccgcctcgggcaaaacgtgcttcattccacgctcaagggcgaggcgcgccgcgactacgtccgcgactgcgtttacttatttctgtgctacacctggcaaacggccatgggcgtgtggcagcaatgcctggaggagcgcaacctaaaggagctgcagaagctgctaaagcaaaacttgaaggacctatggacggccttcaacgagcgctccgtggccgcgcacctggcggacattatcttccccgaacgcctgcttaaaaccctgcaacagggtctgccagacttcaccagtcaaagcatgttgcaaaactttaggaactttatcctagagcgttcaggaattctgcccgccacctgctgtgcgcttcctagcgactttgtgcccattaagtaccgtgaatgccctccgccgctttggggtcactgctaccttctgcagctagccaactaccttgcctaccactccgacatcatggaagacgtgagcggtgacggcctactggagtgtcactgtcgctgcaacctatgcaccccgcaccgctccctggtctgcaattcgcaactgcttagcgaaagtcaaattatcggtacctttgagctgcagggtccctcgcctgacgaaaagtccgcggctccggggttgaaactcactccggggctgtggacgtcggcttaccttcgcaaatttgtacctgaggactaccacgcccacgagattaggttctacgaagaccaatcccgcccgccaaatgcggagcttaccgcctgcgtcattacccagggccacatccttggccaattgcaagccatcaacaaagcccgccaagagtttctgctacgaaagggacggggggtttacctggacccccagtccggcgaggagctcaacccaatccccccgccgccgcagccctatcagcagccgcgggcccttgcttcccaggatggcacccaaaaagaagctgcagctgccgccgccgccacccacggacgaggaggaatactgggacagtcaggcagaggaggttttggacgaggaggaggagatgatggaagactgggacagcctagacgaagcttccgaggccgaagaggtgtcagacgaaacaccgtcaccctcggtcgcattcccctcgccggcgccccagaaattggcaaccgttcccagcatcgctacaacctccgctcctcaggcgccgccggcactgcctgttcgccgacccaaccgtagatgggacaccactggaaccagggccggtaagtctaagcagccgccgccgttagcccaagagcaacaacagcgccaaggctaccgctcgtggcgcgggcacaagaacgccatagttgcttgcttgcaagactgtgggggcaacatctccttcgcccgccgctttcttctctaccatcacggcgtggccttcccccgtaacatcctgcattactaccgtcatctctacagcccctactgcaccggcggcagcggcagcggcagcaacagcagcggtcacacagaagcaaaggcgaccggatagcaagactctgacaaagcccaagaaatccacagcggcggcagcagcaggaggaggagcgctgcgtctggcgcccaacgaacccgtatcgacccgcgagcttagaaataggatttttcccactctgtatgctatatttcaacaaagcaggggccaagaacaagagctgaaaataaaaaacaggtctctgcgctccctcacccgcagctgcctgtatcacaaaagcgaagatcagcttcggcgcacgctggaagacgcggaggctctcttcagcaaatactgcgcgctgactcttaaggactagtttcgcgccctttctcaaatttaagcgcgaaaactacgtcatctccagcggccacacccggcgccagcacctgtcgtcagcgccattatgagcaaggaaattcccacgccctacatgtggagttaccagccacaaatgggacttgcggctggagctgcccaagactactcaacccgaataaactacatgagcgcgggaccccacatgatatcccgggtcaacggaatccgcgcccaccgaaaccgaattctcctcgaacaggcggctattaccaccacacctcgtaataaccttaatccccgtagttggcccgctgccctggtgtaccaggaaagtcccgctcccaccactgtggtacttcccagagacgcccaggccgaagttcagatgactaactcaggggcgcagcttgcgggcggctttcgtcacagggtgcggtcgcccgggcgttttagggcggagtaacttgcatgtattgggaattgtagtttttttaaaatgggaagtgacgtatcgtgggaaaacggaagtgaagatttgaggaagttgtgggttttttggctttcgtttctgggcgtaggttcgcgtgcggttttctgggtgttttttgtggactttaaccgttacgtcattttttagtcctatatatactcgctctgtacttggccctttttacactgtgactgattgagctggtgccgtgtcgagtggtgttttttaataggtttttttactggtaaggctgactgttatggctgccgctgtggaagcgctgtatgttgttctggagcgggagggtgctattttgcctaggcaggagggtttttcaggtgtttatgtgtttttctctcctattaattttgttatacctcctatgggggctgtaatgttgtctctacgcctgcgggtatgtattcccccgggctatttcggtcgctttttagcactgaccgatgttaaccaacctgatgtgtttaccgagtcttacattatgactccggacatgaccgaggaactgtcggtggtgctttttaatcacggtgaccagtttttttacggtcacgccggcatggccgtagtccgtcttatgcttataagggttgtttttcctgttgtaagacaggcttctaatgtttaaatgtttttttttttgttattttattttgtgtttaatgcaggaacccgcagacatgtttgagagaaaaatggtgtctttttctgtggtggttccggaacttacctgcctttatctgcatgagcatgactacgatgtgcttgcttttttgcgcgaggctttgcctgattttttgagcagcaccttgcattttatatcgccgcccatgcaacaagcttacataggggctacgctggttagcatagctccgagtatgcgtgtcataatcagtgtgggttcttttgtcatggttcctggcggggaagtggccgcgctggtccgtgcagacctgcacgattatgttcagctggccctgcgaagggacctacgggatcgcggtatttttgttaatgttccgcttttgaatcttatacaggtctgtgaggaacctgaatttttgcaatcatgattcgctgcttgaggctgaaggtggagggcgctctggagcagatttttacaatggccggacttaatattcgggatttgcttagagacatattgataaggtggcgagatgaaaattatttgggcatggttgaaggtgctggaatgtttatagaggagattcaccctgaagggtttagcctttacgtccacttggacgtgagggcagtttgccttttggaagccattgtgcaacatcttacaaatgccattatctgttctttggctgtagagtttgaccacgccaccggaggggagcgcgttcacttaatagatcttcattttgaggttttggataatcttttggaataaaaaaaaaaaaacatggttcttccagctcttcccgctcctcccgtgtgtgactcgcagaacgaatgtgtaggttggctgggtgtggcttattctgcggtggtggatgttatcagggcagcggcgcatgaaggagtttacatagaacccgaagccagggggcgcctggatgctttgagagagtggatatactacaactactacacagagcgagctaagcgacgagaccggagacgcagatctgtttgtcacgcccgcacctggttttgcttcaggaaatatgactacgtccggcgttccatttggcatgacactacgaccaacacgatctcggttgtctcggcgcactccgtacagtagggatcgcctacctccttttgagacagagacccgcgctaccatactggaggatcatccgctgctgcccgaatgtaacactttgacaatgcacaacgtgagttacgtgcgaggtcttccctgcagtgtgggatttacgctgattcaggaatgggttgttccctgggatatggttctgacgcgggaggagcttgtaatcctgaggaagtgtatgcacgtgtgcctgtgttgtgccaacattgatatcatgacgagcatgatgatccatggttacgagtcctgggctctccactgtcattgttccagtcccggttccctgcagtgcatagccggcgggcaggttttggccagctggtttaggatggtggtggatggcgccatgtttaatcagaggtttatatggtaccgggaggtggtgaattacaacatgccaaaagaggtaatgtttatgtccagcgtgtttatgaggggtcgccacttaatctacctgcgcttgtggtatgatggccacgtgggttctgtggtccccgccatgagctttggatacagcgccttgcactgtgggattttgaacaatattgtggtgctgtgctgcagttactgtgctgatttaagtgagatcagggtgcgctgctgtgcccggaggacaaggcgtctcatgctgcgggcggtgcgaatcatcgctgaggagaccactgccatgttgtattcctgcaggacggagcggcggcggcagcagtttattcgcgcgctgctgcagcaccaccgccctatcctgatgcacgattatgactctacccccatgtaggcgtggacttccccttcgccgcccgttgagcaaccgcaagttggacagcagcctgtggctcagcagctggacagcgacatgaacttaagcgagctgcccggggagtttattaatatcactgatgagcgtttggctcgacaggaaaccgtgtggaatataacacctaagaatatgtctgttacccatgatatgatgctttttaaggccagccggggagaaaggactgtgtactctgtgtgttgggagggaggtggcaggttgaatactagggttctgtgagtttgattaaggtacggtgatcaatataagctatgtggtggtggggctatactactgaatgaaaaatgacttgaaattttctgcaattgaaaaataaacacgttgaaacataacatgcaacaggttcacgattctttattcctgggcaatgtaggagaaggtgtaagagttggtagcaaaagtttcagtggtgtattttccactttcccaggaccatgtaaaagacatagagtaagtgcttacctcgctagtttctgtggattcactagaatcgatgtaggatgttgcccctcctgacgcggtaggagaaggggagggtgccctgcatgtctgccgctgctcttgctcttgccgctgctgaggaggggggcgcatctgccgcagcaccggatgcatctgggaaaagcaaaaaaggggctcgtccctgtttccggaggaatttgcaagcggggtcttgcatgacggggaggcaaacccccgttcgccgcagtccggccggcccgagactcgaaccgggggtcctgcgactcaacccttggaaaataaccctccggctacagggagcgagccacttaatgctttcgctttccagcctaaccgcttacgccgcgcgcggccagtggccaaaaaagctagcgcagcagccgccgcgcctggaaggaagccaaaaggagcgctcccccgttgtctgacgtcgcacacctgggttcgacacgcgggcggtaaccgcatggatcacggcggacggccggatccggggttcgaaccccggtcgtccgccatgatacccttgcgaatttatccaccagaccacggaagagtgcccgcttacaggctctccttttgcacggtctagagcgtcaacgactgcgcacgcctcaccggccagagcgtcccgaccatggagcactttttgccgctgcgcaacatctggaaccgcgtccgcgactttccgcgcgcctccaccaccgccgccggcatcacctggatgtccaggtacatctacggattacgtcgacgtttaaaccatatgatcagctcactcaaaggcggtaatacggttatccacagaatcaggggataacgcaggaaagaacatgtgagcaaaaggccagcaaaaggccaggaaccgtaaaaaggccgcgttgctggcgtttttccataggctccgcccccctgacgagcatcacaaaaatcgacgctcaagtcagaggtggcgaaacccgacaggactataaagataccaggcgtttccccctggaagctccctcgtgcgctctcctgttccgaccctgccgcttaccggatacctgtccgcctttctcccttcgggaagcgtggcgctttctcatagctcacgctgtaggtatctcagttcggtgtaggtcgttcgctccaagctgggctgtgtgcacgaaccccccgttcagcccgaccgctgcgccttatccggtaactatcgtcttgagtccaacccggtaagacacgacttatcgccactggcagcagccactggtaacaggattagcagagcgaggtatgtaggcggtgctacagagttcttgaagtggtggcctaactacggctacactagaagaacagtatttggtatctgcgctctgctgaagccagttaccttcggaaaaagagttggtagctcttgatccggcaaacaaaccaccgctggtagcggtggtttttttgtttgcaagcagcagattacgcgcagaaaaaaaggatctcaagaagatcctttgatcttttctacggggtctgacgctcagtggaacgaaaactcacgttaagggattttggtcatgagattatcaaaaaggatcttcacctagatccttttaaattaaaaatgaagttttaaatcaatctaaagtatatatgagtaaacttggtctgacagttaccaatgcttaatcagtgaggcacctatctcagcgatctgtctatttcgttcatccatagttgcctgactccccgtcgtgtagataactacgatacgggagggcttaccatctggccccagtgctgcaatgataccgcgagacccacgctcaccggctccagatttatcagcaataaaccagccagccggaagggccgagcgcagaagtggtcctgcaactttatccgcctccatccagtctattaattgttgccgggaagctagagtaagtagttcgccagttaatagtttgcgcaacgttgttgccattgctacaggcatcgtggtgtcacgctcgtcgtttggtatggcttcattcagctccggttcccaacgatcaaggcgagttacatgatcccccatgttgtgcaaaaaagcggttagctccttcggtcctccgatcgttgtcagaagtaagttggccgcagtgttatcactcatggttatggcagcactgcataattctcttactgtcatgccatccgtaagatgcttttctgtgactggtgagtactcaaccaagtcattctgagaatagtgtatgcggcgaccgagttgctcttgcccggcgtcaatacgggataataccgcgccacatagcagaactttaaaagtgctcatcattggaaaacgttcttcggggcgaaaactctcaaggatcttaccgctgttgagatccagttcgatgtaacccactcgtgcacccaactgatcttcagcatcttttactttcaccagcgtttctgggtgagcaaaaacaggaaggcaaaatgccgcaaaaaagggaataagggcgacacggaaatgttgaatactcatactcttcctttttcaatattattgaagcatttatcagggttattgtctcatgagcggatacatatttgaatgtatttagaaaaataaacaaataggggttccgcgcacatttccccgaaaagtgccacctaaattgtaagcgttaatattttgttaaaattcgcgttaaatttttgttaaatcagctcattttttaaccaataggccgaaatcggcaaaatcccttataaatcaaaagaatagaccgagatagggttgagtgttgttccagtttggaacaagagtccactattaaagaacgtggactccaacgtcaaagggcgaaaaaccgtctatcagggcgatggcccactacgtgaaccatcaccctaatcaagttttttggggtcgaggtgccgtaaagcactaaatcggaaccctaaagggagcccccgatttagagcttgacggggaaagccggcgaacgtggcgagaaaggaagggaagaaagcgaaaggagcgggcgctagggcgctggcaagtgtagcggtcacgctgcgcgtaaccaccacacccgccgcgcttaatgcgccgctacagggcgcgatggatcc

SEQ ID NO: 23 - DNA, 20 bp, Artificial Sequence
agtaagaccaccgcacagca

SEQ ID NO: 24 - DNA, 20 bp, Artificial Sequence
ccttggtgggtgctactcct

SEQ ID NO: 25 - DNA, 27 bp, Artificial Sequence
cctccaggtctgaagatcagcggccgc

SEQ ID NO: 26 - DNA, 22 bp, Artificial Sequence
gctgtcatctcttgtgggctgt

SEQ ID NO: 27 - DNA, 26 bp, Artificial Sequence
cctgtcatgcccacacaaatctctcc

SEQ ID NO: 28 - DNA, 21 bp, Artificial Sequence
actcatgggagctgctggttc